European Patent Application EP 4 768 500 A1, published July 1, 2026. Title: ADENO-ASSOCIATED VIRUS VARIANT. Applicant: AAVATAR THERAPEUTICS CO., LTD. Application KR PCT/KR2024/015929, filed October 18, 2024. The sequence listing filed with the application follows.

SEQUENCE LISTING (156 sequences)

SEQ ID NO: 1 - protein, 735 aa, synthetic construct [sequence omitted]

SEQ ID NO: 2 - protein, 735 aa, synthetic construct
  source 1..735: note = Amino acid sequence of VP1 variant
MAADGYLPDWLEDTLSEGIRQWWKLKPGPPPPKPAERHKDDSRGLVLPGYKYLGPFNGLDKGEPVNEADAAALEHDKAYDRQLDSGDNPYLKYNHADAEFQERLKEDTSFGGNLGRAVFQAKKRVLEPLGLVEEPVKTAPGKKRPVEHSPVEPDSSSGTGKAGQQPARKRLNFGQTGDADSVPDPQPLGQPPAAPSGLGTNTMATGSGAPMADNNEGADGVGNSSGNWHCDSTWMGDRVITTSTRTWALPTYNNHLYKQISSQSGASNDNHYFGYSTPWGYFDFNRFHCHFSPRDWQRLINNNWGFRPKRLNFKLFNIQVKEVTQNDGTTTIANNLTSTVQVFTDSEYQLPYVLGSAHQGCLPPFPADVFMVPQYGYLTLNNGSQAVGRSSFYCLEYFPSQMLRTGNNFTFSYTFEDVPFHSSYAHSQSLDRLMNPLIDQYLYYLSRTNTPSGTTTQSRLQFSQAGASDIRDQSRNWLPGPCYRQQRVSKTSADNNNSEYSWTGATKYHLNGRDSLVNPGPAMASHKDDEEKFFPQSGVLIFGKQGSEKTNVDIEKVMITDEEEIAATNPVATESYGEVATNLQRGNVQAATADVNTQGVLPGMVWQDRDVYLQGPIWAKIPHTDGHFHPSPLMGGFGLKHPPPQILIKNTPVPANPSTTFSAAKFASFITQYSTGQVSVEIEWELQKENSKRWNPEIQYTSNYNKSVNVDFTVDTNGVYSEPRPIGTRYLTRNL

SEQ ID NO: 3 - protein, 735 aa, synthetic construct
  source 1..735: note = Amino acid sequence of VP1 variant
MAADGYLPDWLEDTLSEGIRQWWKLKPGPPPPKPAERHKDDSRGLVLPGYKYLGPFNGLDKGEPVNEADAAALEHDKAYDRQLDSGDNPYLKYNHADAEFQERLKEDTSFGGNLGRAVFQAKKRVLEPLGLVEEPVKTAPGKKRPVEHSPVEPDSSSGTGKAGQQPARKRLNFGQTGDADSVPDPQPLGQPPAAPSGLGTNTMATGSGAPMADNNEGADGVGNSSGNWHCDSTWMGDRVITTSTRTWALPTYNNHLYKQISSQSGASNDNHYFGYSTPWGYFDFNRFHCHFSPRDWQRLINNNWGFRPKRLNFKLFNIQVKEVTQNDGTTTIANNLTSTVQVFTDSEYQLPYVLGSAHQGCLPPFPADVFMVPQYGYLTLNNGSQAVGRSSFYCLEYFPSQMLRTGNNFTFSYTFEDVPFHSSYAHSQSLDRLMNPLIDQYLYYLSRTNTPSGTTTQSRLQFSQAGASDIRDQSRNWLPGPCYRQQRVSKTSADNNNSEYSWTGATKYHLNGRDSLVNPGPAMASHKDDEEKFFPQSGVLIFGKQGSEKTNVDIEKVMITDEQEVAATNPVATESWGSVSTNLQRGNTQAATADVNTQGVLPGMVWQDRDVYLQGPIWAKIPHTDGHFHPSPLMGGFGLKHPPPQILIKNTPVPANPSTTFSAAKFASFITQYSTGQVSVEIEWELQKENSKRWNPEIQYTSNYNKSVNVDFTVDTNGVYSEPRPIGTRYLTRNL

SEQ ID NO: 4 - protein, 735 aa, synthetic construct
  source 1..735: note = Amino acid sequence of VP1 variant
MAADGYLPDWLEDTLSEGIRQWWKLKPGPPPPKPAERHKDDSRGLVLPGYKYLGPFNGLDKGEPVNEADAAALEHDKAYDRQLDSGDNPYLKYNHADAEFQERLKEDTSFGGNLGRAVFQAKKRVLEPLGLVEEPVKTAPGKKRPVEHSPVEPDSSSGTGKAGQQPARKRLNFGQTGDADSVPDPQPLGQPPAAPSGLGTNTMATGSGAPMADNNEGADGVGNSSGNWHCDSTWMGDRVITTSTRTWALPTYNNHLYKQISSQSGASNDNHYFGYSTPWGYFDFNRFHCHFSPRDWQRLINNNWGFRPKRLNFKLFNIQVKEVTQNDGTTTIANNLTSTVQVFTDSEYQLPYVLGSAHQGCLPPFPADVFMVPQYGYLTLNNGSQAVGRSSFYCLEYFPSQMLRTGNNFTFSYTFEDVPFHSSYAHSQSLDRLMNPLIDQYLYYLSRTNTPSGTTTQSRLQFSQAGASDIRDQSRNWLPGPCYRQQRVSKTSADNNNSEYSWTGATKYHLNGRDSLVNPGPAMASHKDDEEKFFPQSGVLIFGKQGSEKTNVDIEKVMITDESEIRTTNPIATEQWGSVSTNLQNGNRQAATADVNTQGVLPGMVWQDRDVYLQGPIWAKIPHTDGHFHPSPLMGGFGLKHPPPQILIKNTPVPANPSTTFSAAKFASFITQYSTGQVSVEIEWELQKENSKRWNPEIQYTSNYNKSVNVDFTVDTNGVYSEPRPIGTRYLTRNL

SEQ ID NO: 5 - protein, 735 aa, synthetic construct
  source 1..735: note = Amino acid sequence of VP1 variant
MAADGYLPDWLEDTLSEGIRQWWKLKPGPPPPKPAERHKDDSRGLVLPGYKYLGPFNGLDKGEPVNEADAAALEHDKAYDRQLDSGDNPYLKYNHADAEFQERLKEDTSFGGNLGRAVFQAKKRVLEPLGLVEEPVKTAPGKKRPVEHSPVEPDSSSGTGKAGQQPARKRLNFGQTGDADSVPDPQPLGQPPAAPSGLGTNTMATGSGAPMADNNEGADGVGNSSGNWHCDSTWMGDRVITTSTRTWALPTYNNHLYKQISSQSGASNDNHYFGYSTPWGYFDFNRFHCHFSPRDWQRLINNNWGFRPKRLNFKLFNIQVKEVTQNDGTTTIANNLTSTVQVFTDSEYQLPYVLGSAHQGCLPPFPADVFMVPQYGYLTLNNGSQAVGRSSFYCLEYFPSQMLRTGNNFTFSYTFEDVPFHSSYAHSQSLDRLMNPLIDQYLYYLSRTNTPSGTTTQSRLQFSQAGASDIRDQSRNWLPGPCYRQQRVSKTSADNNNSEYSWTGATKYHLNGRDSLVNPGPAMASHKDDEEKFFPQSGVLIFGKQGSEKTNVDIEKVMITDEEEIATTNPVATEQWGSVSTNLQRGATQAATADVNTQGVLPGMVWQDRDVYLQGPIWAKIPHTDGHFHPSPLMGGFGLKHPPPQILIKNTPVPANPSTTFSAAKFASFITQYSTGQVSVEIEWELQKENSKRWNPEIQYTSNYNKSVNVDFTVDTNGVYSEPRPIGTRYLTRNL

SEQ ID NO: 6 - protein, 735 aa, synthetic construct
  source 1..735: note = Amino acid sequence of VP1 variant
MAADGYLPDWLEDTLSEGIRQWWKLKPGPPPPKPAERHKDDSRGLVLPGYKYLGPFNGLDKGEPVNEADAAALEHDKAYDRQLDSGDNPYLKYNHADAEFQERLKEDTSFGGNLGRAVFQAKKRVLEPLGLVEEPVKTAPGKKRPVEHSPVEPDSSSGTGKAGQQPARKRLNFGQTGDADSVPDPQPLGQPPAAPSGLGTNTMATGSGAPMADNNEGADGVGNSSGNWHCDSTWMGDRVITTSTRTWALPTYNNHLYKQISSQSGASNDNHYFGYSTPWGYFDFNRFHCHFSPRDWQRLINNNWGFRPKRLNFKLFNIQVKEVTQNDGTTTIANNLTSTVQVFTDSEYQLPYVLGSAHQGCLPPFPADVFMVPQYGYLTLNNGSQAVGRSSFYCLEYFPSQMLRTGNNFTFSYTFEDVPFHSSYAHSQSLDRLMNPLIDQYLYYLSRTNTPSGTTTQSRLQFSQAGASDIRDQSRNWLPGPCYRQQRVSKTSADNNNSEYSWTGATKYHLNGRDSLVNPGPAMASHKDDEEKFFPQSGVLIFGKQGSEKTNVDIEKVMITDESEIATTNPVATESYGEVSTNLQRNPVQAATADVNTQGVLPGMVWQDRDVYLQGPIWAKIPHTDGHFHPSPLMGGFGLKHPPPQILIKNTPVPANPSTTFSAAKFASFITQYSTGQVSVEIEWELQKENSKRWNPEIQYTSNYNKSVNVDFTVDTNGVYSEPRPIGTRYLTRNL

SEQ ID NO: 7 - protein, 735 aa, synthetic construct
  source 1..735: note = Amino acid sequence of VP1 variant
MAADGYLPDWLEDTLSEGIRQWWKLKPGPPPPKPAERHKDDSRGLVLPGYKYLGPFNGLDKGEPVNEADAAALEHDKAYDRQLDSGDNPYLKYNHADAEFQERLKEDTSFGGNLGRAVFQAKKRVLEPLGLVEEPVKTAPGKKRPVEHSPVEPDSSSGTGKAGQQPARKRLNFGQTGDADSVPDPQPLGQPPAAPSGLGTNTMATGSGAPMADNNEGADGVGNSSGNWHCDSTWMGDRVITTSTRTWALPTYNNHLYKQISSQSGASNDNHYFGYSTPWGYFDFNRFHCHFSPRDWQRLINNNWGFRPKRLNFKLFNIQVKEVTQNDGTTTIANNLTSTVQVFTDSEYQLPYVLGSAHQGCLPPFPADVFMVPQYGYLTLNNGSQAVGRSSFYCLEYFPSQMLRTGNNFTFSYTFEDVPFHSSYAHSQSLDRLMNPLIDQYLYYLSRTNTPSGTTTQSRLQFSQAGASDIRDQSRNWLPGPCYRQQRVSKTSADNNNSEYSWTGATKYHLNGRDSLVNPGPAMASHKDDEEKFFPQSGVLIFGKQGSEKTNVDIEKVMITDEEEIRTTNPVAYEQYGVVATNLQNSNAQAATADVNTQGVLPGMVWQDRDVYLQGPIWAKIPHTDGHFHPSPLMGGFGLKHPPPQILIKNTPVPANPSTTFSAAKFASFITQYSTGQVSVEIEWELQKENSKRWNPEIQYTSNYNKSVNVDFTVDTNGVYSEPRPIGTRYLTRNL

SEQ ID NO: 8 - protein, 735 aa, synthetic construct
  source 1..735: note = Amino acid sequence of VP1 variant
MAADGYLPDWLEDTLSEGIRQWWKLKPGPPPPKPAERHKDDSRGLVLPGYKYLGPFNGLDKGEPVNEADAAALEHDKAYDRQLDSGDNPYLKYNHADAEFQERLKEDTSFGGNLGRAVFQAKKRVLEPLGLVEEPVKTAPGKKRPVEHSPVEPDSSSGTGKAGQQPARKRLNFGQTGDADSVPDPQPLGQPPAAPSGLGTNTMATGSGAPMADNNEGADGVGNSSGNWHCDSTWMGDRVITTSTRTWALPTYNNHLYKQISSQSGASNDNHYFGYSTPWGYFDFNRFHCHFSPRDWQRLINNNWGFRPKRLNFKLFNIQVKEVTQNDGTTTIANNLTSTVQVFTDSEYQLPYVLGSAHQGCLPPFPADVFMVPQYGYLTLNNGSQAVGRSSFYCLEYFPSQMLRTGNNFTFSYTFEDVPFHSSYAHSQSLDRLMNPLIDQYLYYLSRTNTPSGTTTQSRLQFSQAGASDIRDQSRNWLPGPCYRQQRVSKTSADNNNSEYSWTGATKYHLNGRDSLVNPGPAMASHKDDEEKFFPQSGVLIFGKQGSEKTNVDIEKVMITDEAEIATTNPVAAEQYGEVSTNLQNGNRQAATADVNTQGVLPGMVWQDRDVYLQGPIWAKIPHTDGHFHPSPLMGGFGLKHPPPQILIKNTPVPANPSTTFSAAKFASFITQYSTGQVSVEIEWELQKENSKRWNPEIQYTSNYNKSVNVDFTVDTNGVYSEPRPIGTRYLTRNL

SEQ ID NO: 9 - protein, 735 aa, synthetic construct
  source 1..735: note = Amino acid sequence of VP1 variant
MAADGYLPDWLEDTLSEGIRQWWKLKPGPPPPKPAERHKDDSRGLVLPGYKYLGPFNGLDKGEPVNEADAAALEHDKAYDRQLDSGDNPYLKYNHADAEFQERLKEDTSFGGNLGRAVFQAKKRVLEPLGLVEEPVKTAPGKKRPVEHSPVEPDSSSGTGKAGQQPARKRLNFGQTGDADSVPDPQPLGQPPAAPSGLGTNTMATGSGAPMADNNEGADGVGNSSGNWHCDSTWMGDRVITTSTRTWALPTYNNHLYKQISSQSGASNDNHYFGYSTPWGYFDFNRFHCHFSPRDWQRLINNNWGFRPKRLNFKLFNIQVKEVTQNDGTTTIANNLTSTVQVFTDSEYQLPYVLGSAHQGCLPPFPADVFMVPQYGYLTLNNGSQAVGRSSFYCLEYFPSQMLRTGNNFTFSYTFEDVPFHSSYAHSQSLDRLMNPLIDQYLYYLSRTNTPSGTTTQSRLQFSQAGASDIRDQSRNWLPGPCYRQQRVSKTSADNNNSEYSWTGATKYHLNGRDSLVNPGPAMASHKDDEEKFFPQSGVLIFGKQGSEKTNVDIEKVMITDEQEVAATNPVATEHYGQVATNLQTGNRQAATADVNTQGVLPGMVWQDRDVYLQGPIWAKIPHTDGHFHPSPLMGGFGLKHPPPQILIKNTPVPANPSTTFSAAKFASFITQYSTGQVSVEIEWELQKENSKRWNPEIQYTSNYNKSVNVDFTVDTNGVYSEPRPIGTRYLTRNL

SEQ ID NO: 10 - protein, 735 aa, synthetic construct
  source 1..735: note = Amino acid sequence of VP1 variant
MAADGYLPDWLEDTLSEGIRQWWKLKPGPPPPKPAERHKDDSRGLVLPGYKYLGPFNGLDKGEPVNEADAAALEHDKAYDRQLDSGDNPYLKYNHADAEFQERLKEDTSFGGNLGRAVFQAKKRVLEPLGLVEEPVKTAPGKKRPVEHSPVEPDSSSGTGKAGQQPARKRLNFGQTGDADSVPDPQPLGQPPAAPSGLGTNTMATGSGAPMADNNEGADGVGNSSGNWHCDSTWMGDRVITTSTRTWALPTYNNHLYKQISSQSGASNDNHYFGYSTPWGYFDFNRFHCHFSPRDWQRLINNNWGFRPKRLNFKLFNIQVKEVTQNDGTTTIANNLTSTVQVFTDSEYQLPYVLGSAHQGCLPPFPADVFMVPQYGYLTLNNGSQAVGRSSFYCLEYFPSQMLRTGNNFTFSYTFEDVPFHSSYAHSQSLDRLMNPLIDQYLYYLSRTNTPSGTTTQSRLQFSQAGASDIRDQSRNWLPGPCYRQQRVSKTSADNNNSEYSWTGATKYHLNGRDSLVNPGPAMASHKDDEEKFFPQSGVLIFGKQGSEKTNVDIEKVMITDEEEINTTNPVYTEQYGSVSTNLQRGNIQAATADVNTQGVLPGMVWQDRDVYLQGPIWAKIPHTDGHFHPSPLMGGFGLKHPPPQILIKNTPVPANPSTTFSAAKFASFITQYSTGQVSVEIEWELQKENSKRWNPEIQYTSNYNKSVNVDFTVDTNGVYSEPRPIGTRYLTRNL

SEQ ID NO: 11 - protein, 735 aa, synthetic construct
  source 1..735: note = Amino acid sequence of VP1 variant
MAADGYLPDWLEDTLSEGIRQWWKLKPGPPPPKPAERHKDDSRGLVLPGYKYLGPFNGLDKGEPVNEADAAALEHDKAYDRQLDSGDNPYLKYNHADAEFQERLKEDTSFGGNLGRAVFQAKKRVLEPLGLVEEPVKTAPGKKRPVEHSPVEPDSSSGTGKAGQQPARKRLNFGQTGDADSVPDPQPLGQPPAAPSGLGTNTMATGSGAPMADNNEGADGVGNSSGNWHCDSTWMGDRVITTSTRTWALPTYNNHLYKQISSQSGASNDNHYFGYSTPWGYFDFNRFHCHFSPRDWQRLINNNWGFRPKRLNFKLFNIQVKEVTQNDGTTTIANNLTSTVQVFTDSEYQLPYVLGSAHQGCLPPFPADVFMVPQYGYLTLNNGSQAVGRSSFYCLEYFPSQMLRTGNNFTFSYTFEDVPFHSSYAHSQSLDRLMNPLIDQYLYYLSRTNTPSGTTTQSRLQFSQAGASDIRDQSRNWLPGPCYRQQRVSKTSADNNNSEYSWTGATKYHLNGRDSLVNPGPAMASHKDDEEKFFPQSGVLIFGKQGSEKTNVDIEKVMITDEQEVAATNPVADEQYGVVATNLQRGNVQAATADVNTQGVLPGMVWQDRDVYLQGPIWAKIPHTDGHFHPSPLMGGFGLKHPPPQILIKNTPVPANPSTTFSAAKFASFITQYSTGQVSVEIEWELQKENSKRWNPEIQYTSNYNKSVNVDFTVDTNGVYSEPRPIGTRYLTRNL

SEQ ID NO: 12 - protein, 735 aa, synthetic construct
  source 1..735: note = Amino acid sequence of VP1 variant
MAADGYLPDWLEDTLSEGIRQWWKLKPGPPPPKPAERHKDDSRGLVLPGYKYLGPFNGLDKGEPVNEADAAALEHDKAYDRQLDSGDNPYLKYNHADAEFQERLKEDTSFGGNLGRAVFQAKKRVLEPLGLVEEPVKTAPGKKRPVEHSPVEPDSSSGTGKAGQQPARKRLNFGQTGDADSVPDPQPLGQPPAAPSGLGTNTMATGSGAPMADNNEGADGVGNSSGNWHCDSTWMGDRVITTSTRTWALPTYNNHLYKQISSQSGASNDNHYFGYSTPWGYFDFNRFHCHFSPRDWQRLINNNWGFRPKRLNFKLFNIQVKEVTQNDGTTTIANNLTSTVQVFTDSEYQLPYVLGSAHQGCLPPFPADVFMVPQYGYLTLNNGSQAVGRSSFYCLEYFPSQMLRTGNNFTFSYTFEDVPFHSSYAHSQSLDRLMNPLIDQYLYYLSRTNTPSGTTTQSRLQFSQAGASDIRDQSRNWLPGPCYRQQRVSKTSADNNNSEYSWTGATKYHLNGRDSLVNPGPAMASHKDDEEKFFPQSGVLIFGKQGSEKTNVDIEKVMITDESEIAATNPVATEQWGSVATNRQRGETQAATADVNTQGVLPGMVWQDRDVYLQGPIWAKIPHTDGHFHPSPLMGGFGLKHPPPQILIKNTPVPANPSTTFSAAKFASFITQYSTGQVSVEIEWELQKENSKRWNPEIQYTSNYNKSVNVDFTVDTNGVYSEPRPIGTRYLTRNL

SEQ ID NO: 13 - protein, 735 aa, synthetic construct
  source 1..735: note = Amino acid sequence of VP1 variant
MAADGYLPDWLEDTLSEGIRQWWKLKPGPPPPKPAERHKDDSRGLVLPGYKYLGPFNGLDKGEPVNEADAAALEHDKAYDRQLDSGDNPYLKYNHADAEFQERLKEDTSFGGNLGRAVFQAKKRVLEPLGLVEEPVKTAPGKKRPVEHSPVEPDSSSGTGKAGQQPARKRLNFGQTGDADSVPDPQPLGQPPAAPSGLGTNTMATGSGAPMADNNEGADGVGNSSGNWHCDSTWMGDRVITTSTRTWALPTYNNHLYKQISSQSGASNDNHYFGYSTPWGYFDFNRFHCHFSPRDWQRLINNNWGFRPKRLNFKLFNIQVKEVTQNDGTTTIANNLTSTVQVFTDSEYQLPYVLGSAHQGCLPPFPADVFMVPQYGYLTLNNGSQAVGRSSFYCLEYFPSQMLRTGNNFTFSYTFEDVPFHSSYAHSQSLDRLMNPLIDQYLYYLSRTNTPSGTTTQSRLQFSQAGASDIRDQSRNWLPGPCYRQQRVSKTSADNNNSEYSWTGATKYHLNGRDSLVNPGPAMASHKDDEEKFFPQSGVLIFGKQGSEKTNVDIEKVMITDEQEVAATNPVATEQWGEVSTNLQRSTTQAATADVNTQGVLPGMVWQDRDVYLQGPIWAKIPHTDGHFHPSPLMGGFGLKHPPPQILIKNTPVPANPSTTFSAAKFASFITQYSTGQVSVEIEWELQKENSKRWNPEIQYTSNYNKSVNVDFTVDTNGVYSEPRPIGTRYLTRNL

SEQ ID NO: 14 - protein, 735 aa, synthetic construct
  source 1..735: note = Amino acid sequence of VP1 variant
MAADGYLPDWLEDTLSEGIRQWWKLKPGPPPPKPAERHKDDSRGLVLPGYKYLGPFNGLDKGEPVNEADAAALEHDKAYDRQLDSGDNPYLKYNHADAEFQERLKEDTSFGGNLGRAVFQAKKRVLEPLGLVEEPVKTAPGKKRPVEHSPVEPDSSSGTGKAGQQPARKRLNFGQTGDADSVPDPQPLGQPPAAPSGLGTNTMATGSGAPMADNNEGADGVGNSSGNWHCDSTWMGDRVITTSTRTWALPTYNNHLYKQISSQSGASNDNHYFGYSTPWGYFDFNRFHCHFSPRDWQRLINNNWGFRPKRLNFKLFNIQVKEVTQNDGTTTIANNLTSTVQVFTDSEYQLPYVLGSAHQGCLPPFPADVFMVPQYGYLTLNNGSQAVGRSSFYCLEYFPSQMLRTGNNFTFSYTFEDVPFHSSYAHSQSLDRLMNPLIDQYLYYLSRTNTPSGTTTQSRLQFSQAGASDIRDQSRNWLPGPCYRQQRVSKTSADNNNSEYSWTGATKYHLNGRDSLVNPGPAMASHKDDEEKFFPQSGVLIFGKQGSEKTNVDIEKVMITQESEIAATNPVATEQWGVVATNLQNGTRQAATADVNTQGVLPGMVWQDRDVYLQGPIWAKIPHTDGHFHPSPLMGGFGLKHPPPQILIKNTPVPANPSTTFSAAKFASFITQYSTGQVSVEIEWELQKENSKRWNPEIQYTSNYNKSVNVDFTVDTNGVYSEPRPIGTRYLTRNL

SEQ ID NO: 15 - protein, 735 aa, synthetic construct
  source 1..735: note = Amino acid sequence of VP1 variant
MAADGYLPDWLEDTLSEGIRQWWKLKPGPPPPKPAERHKDDSRGLVLPGYKYLGPFNGLDKGEPVNEADAAALEHDKAYDRQLDSGDNPYLKYNHADAEFQERLKEDTSFGGNLGRAVFQAKKRVLEPLGLVEEPVKTAPGKKRPVEHSPVEPDSSSGTGKAGQQPARKRLNFGQTGDADSVPDPQPLGQPPAAPSGLGTNTMATGSGAPMADNNEGADGVGNSSGNWHCDSTWMGDRVITTSTRTWALPTYNNHLYKQISSQSGASNDNHYFGYSTPWGYFDFNRFHCHFSPRDWQRLINNNWGFRPKRLNFKLFNIQVKEVTQNDGTTTIANNLTSTVQVFTDSEYQLPYVLGSAHQGCLPPFPADVFMVPQYGYLTLNNGSQAVGRSSFYCLEYFPSQMLRTGNNFTFSYTFEDVPFHSSYAHSQSLDRLMNPLIDQYLYYLSRTNTPSGTTTQSRLQFSQAGASDIRDQSRNWLPGPCYRQQRVSKTSADNNNSEYSWTGATKYHLNGRDSLVNPGPAMASHKDDEEKFFPQSGVLIFGKQGSEKTNVDIEKVMITDESEVAATNPVATEQWGEVSTNNQRGTTQAATADVNTQGVLPGMVWQDRDVYLQGPIWAKIPHTDGHFHPSPLMGGFGLKHPPPQILIKNTPVPANPSTTFSAAKFASFITQYSTGQVSVEIEWELQKENSKRWNPEIQYTSNYNKSVNVDFTVDTNGVYSEPRPIGTRYLTRNL

SEQ ID NO: 16 - protein, 735 aa, synthetic construct
  source 1..735: note = Amino acid sequence of VP1 variant
MAADGYLPDWLEDTLSEGIRQWWKLKPGPPPPKPAERHKDDSRGLVLPGYKYLGPFNGLDKGEPVNEADAAALEHDKAYDRQLDSGDNPYLKYNHADAEFQERLKEDTSFGGNLGRAVFQAKKRVLEPLGLVEEPVKTAPGKKRPVEHSPVEPDSSSGTGKAGQQPARKRLNFGQTGDADSVPDPQPLGQPPAAPSGLGTNTMATGSGAPMADNNEGADGVGNSSGNWHCDSTWMGDRVITTSTRTWALPTYNNHLYKQISSQSGASNDNHYFGYSTPWGYFDFNRFHCHFSPRDWQRLINNNWGFRPKRLNFKLFNIQVKEVTQNDGTTTIANNLTSTVQVFTDSEYQLPYVLGSAHQGCLPPFPADVFMVPQYGYLTLNNGSQAVGRSSFYCLEYFPSQMLRTGNNFTFSYTFEDVPFHSSYAHSQSLDRLMNPLIDQYLYYLSRTNTPSGTTTQSRLQFSQAGASDIRDQSRNWLPGPCYRQQRVSKTSADNNNSEYSWTGATKYHLNGRDSLVNPGPAMASHKDDEEKFFPQSGVLIFGKQGSEKTNVDIEKVMITDEEEIRTTNPVATEQYGSVSTNIQHGNRQAATADVNTQGVLPGMVWQDRDVYLQGPIWAKIPHTDGHFHPSPLMGGFGLKHPPPQILIKNTPVPANPSTTFSAAKFASFITQYSTGQVSVEIEWELQKENSKRWNPEIQYTSNYNKSVNVDFTVDTNGVYSEPRPIGTRYLTRNL

SEQ ID NO: 17 - protein, 735 aa, synthetic construct
  source 1..735: note = Amino acid sequence of VP1 variant
MAADGYLPDWLEDTLSEGIRQWWKLKPGPPPPKPAERHKDDSRGLVLPGYKYLGPFNGLDKGEPVNEADAAALEHDKAYDRQLDSGDNPYLKYNHADAEFQERLKEDTSFGGNLGRAVFQAKKRVLEPLGLVEEPVKTAPGKKRPVEHSPVEPDSSSGTGKAGQQPARKRLNFGQTGDADSVPDPQPLGQPPAAPSGLGTNTMATGSGAPMADNNEGADGVGNSSGNWHCDSTWMGDRVITTSTRTWALPTYNNHLYKQISSQSGASNDNHYFGYSTPWGYFDFNRFHCHFSPRDWQRLINNNWGFRPKRLNFKLFNIQVKEVTQNDGTTTIANNLTSTVQVFTDSEYQLPYVLGSAHQGCLPPFPADVFMVPQYGYLTLNNGSQAVGRSSFYCLEYFPSQMLRTGNNFTFSYTFEDVPFHSSYAHSQSLDRLMNPLIDQYLYYLSRTNTPSGTTTQSRLQFSQAGASDIRDQSRNWLPGPCYRQQRVSKTSADNNNSEYSWTGATKYHLNGRDSLVNPGPAMASHKDDEEKFFPQSGVLIFGKQGSEKTNVDIEKVMITDEEEIRTTNPVATEQYGSVSTWLQRGNRQAATADVNTQGVLPGMVWQDRDVYLQGPIWAKIPHTDGHFHPSPLMGGFGLKHPPPQILIKNTPVPANPSTTFSAAKFASFITQYSTGQVSVEIEWELQKENSKRWNPEIQYTSNYNKSVNVDFTVDTNGVYSEPRPIGTRYLTRNL

SEQ ID NO: 18 - protein, 735 aa, synthetic construct
  source 1..735: note = Amino acid sequence of VP1 variant
MAADGYLPDWLEDTLSEGIRQWWKLKPGPPPPKPAERHKDDSRGLVLPGYKYLGPFNGLDKGEPVNEADAAALEHDKAYDRQLDSGDNPYLKYNHADAEFQERLKEDTSFGGNLGRAVFQAKKRVLEPLGLVEEPVKTAPGKKRPVEHSPVEPDSSSGTGKAGQQPARKRLNFGQTGDADSVPDPQPLGQPPAAPSGLGTNTMATGSGAPMADNNEGADGVGNSSGNWHCDSTWMGDRVITTSTRTWALPTYNNHLYKQISSQSGASNDNHYFGYSTPWGYFDFNRFHCHFSPRDWQRLINNNWGFRPKRLNFKLFNIQVKEVTQNDGTTTIANNLTSTVQVFTDSEYQLPYVLGSAHQGCLPPFPADVFMVPQYGYLTLNNGSQAVGRSSFYCLEYFPSQMLRTGNNFTFSYTFEDVPFHSSYAHSQSLDRLMNPLIDQYLYYLSRTNTPSGTTTQSRLQFSQAGASDIRDQSRNWLPGPCYRQQRVSKTSADNNNSEYSWTGATKYHLNGRDSLVNPGPAMASHKDDEEKFFPQSGVLIFGKQGSEKTNVDIEKVMITDEQEIAATNPVATEQYGEVSTNLQNQNRQAATADVNTQGVLPGMVWQDRDVYLQGPIWAKIPHTDGHFHPSPLMGGFGLKHPPPQILIKNTPVPANPSTTFSAAKFASFITQYSTGQVSVEIEWELQKENSKRWNPEIQYTSNYNKSVNVDFTVDTNGVYSEPRPIGTRYLTRNL

SEQ ID NO: 19 - protein, 735 aa, synthetic construct
  source 1..735: note = Amino acid sequence of VP1 variant
MAADGYLPDWLEDTLSEGIRQWWKLKPGPPPPKPAERHKDDSRGLVLPGYKYLGPFNGLDKGEPVNEADAAALEHDKAYDRQLDSGDNPYLKYNHADAEFQERLKEDTSFGGNLGRAVFQAKKRVLEPLGLVEEPVKTAPGKKRPVEHSPVEPDSSSGTGKAGQQPARKRLNFGQTGDADSVPDPQPLGQPPAAPSGLGTNTMATGSGAPMADNNEGADGVGNSSGNWHCDSTWMGDRVITTSTRTWALPTYNNHLYKQISSQSGASNDNHYFGYSTPWGYFDFNRFHCHFSPRDWQRLINNNWGFRPKRLNFKLFNIQVKEVTQNDGTTTIANNLTSTVQVFTDSEYQLPYVLGSAHQGCLPPFPADVFMVPQYGYLTLNNGSQAVGRSSFYCLEYFPSQMLRTGNNFTFSYTFEDVPFHSSYAHSQSLDRLMNPLIDQYLYYLSRTNTPSGTTTQSRLQFSQAGASDIRDQSRNWLPGPCYRQQRVSKTSADNNNSEYSWTGATKYHLNGRDSLVNPGPAMASHKDDEEKFFPQSGVLIFGKQGSEKTNVDIEKVMITQESEIAATNPVATEQWGEVATNLQRGTTQAATADVNTQGVLPGMVWQDRDVYLQGPIWAKIPHTDGHFHPSPLMGGFGLKHPPPQILIKNTPVPANPSTTFSAAKFASFITQYSTGQVSVEIEWELQKENSKRWNPEIQYTSNYNKSVNVDFTVDTNGVYSEPRPIGTRYLTRNL

SEQ ID NO: 20 - protein, 735 aa, synthetic construct
  source 1..735: note = Amino acid sequence of VP1 variant
MAADGYLPDWLEDTLSEGIRQWWKLKPGPPPPKPAERHKDDSRGLVLPGYKYLGPFNGLDKGEPVNEADAAALEHDKAYDRQLDSGDNPYLKYNHADAEFQERLKEDTSFGGNLGRAVFQAKKRVLEPLGLVEEPVKTAPGKKRPVEHSPVEPDSSSGTGKAGQQPARKRLNFGQTGDADSVPDPQPLGQPPAAPSGLGTNTMATGSGAPMADNNEGADGVGNSSGNWHCDSTWMGDRVITTSTRTWALPTYNNHLYKQISSQSGASNDNHYFGYSTPWGYFDFNRFHCHFSPRDWQRLINNNWGFRPKRLNFKLFNIQVKEVTQNDGTTTIANNLTSTVQVFTDSEYQLPYVLGSAHQGCLPPFPADVFMVPQYGYLTLNNGSQAVGRSSFYCLEYFPSQMLRTGNNFTFSYTFEDVPFHSSYAHSQSLDRLMNPLIDQYLYYLSRTNTPSGTTTQSRLQFSQAGASDIRDQSRNWLPGPCYRQQRVSKTSADNNNSEYSWTGATKYHLNGRDSLVNPGPAMASHKDDEEKFFPQSGVLIFGKQGSEKTNVDIEKVMITDEWEIRTTNPVATEQYGSVSTNLQRLNRQAATADVNTQGVLPGMVWQDRDVYLQGPIWAKIPHTDGHFHPSPLMGGFGLKHPPPQILIKNTPVPANPSTTFSAAKFASFITQYSTGQVSVEIEWELQKENSKRWNPEIQYTSNYNKSVNVDFTVDTNGVYSEPRPIGTRYLTRNL

SEQ ID NO: 21 - protein, 735 aa, synthetic construct
  source 1..735: note = Amino acid sequence of VP1 variant
MAADGYLPDWLEDTLSEGIRQWWKLKPGPPPPKPAERHKDDSRGLVLPGYKYLGPFNGLDKGEPVNEADAAALEHDKAYDRQLDSGDNPYLKYNHADAEFQERLKEDTSFGGNLGRAVFQAKKRVLEPLGLVEEPVKTAPGKKRPVEHSPVEPDSSSGTGKAGQQPARKRLNFGQTGDADSVPDPQPLGQPPAAPSGLGTNTMATGSGAPMADNNEGADGVGNSSGNWHCDSTWMGDRVITTSTRTWALPTYNNHLYKQISSQSGASNDNHYFGYSTPWGYFDFNRFHCHFSPRDWQRLINNNWGFRPKRLNFKLFNIQVKEVTQNDGTTTIANNLTSTVQVFTDSEYQLPYVLGSAHQGCLPPFPADVFMVPQYGYLTLNNGSQAVGRSSFYCLEYFPSQMLRTGNNFTFSYTFEDVPFHSSYAHSQSLDRLMNPLIDQYLYYLSRTNTPSGTTTQSRLQFSQAGASDIRDQSRNWLPGPCYRQQRVSKTSADNNNSEYSWTGATKYHLNGRDSLVNPGPAMASHKDDEEKFFPQSGVLIFGKQGSEKTNVDIEKVMITDEAEIAATNPVATEQWGEVSTNTQNGARQAATADVNTQGVLPGMVWQDRDVYLQGPIWAKIPHTDGHFHPSPLMGGFGLKHPPPQILIKNTPVPANPSTTFSAAKFASFITQYSTGQVSVEIEWELQKENSKRWNPEIQYTSNYNKSVNVDFTVDTNGVYSEPRPIGTRYLTRNL

SEQ ID NO: 22 - protein, 735 aa, synthetic construct
  source 1..735: note = Amino acid sequence of VP1 variant
MAADGYLPDWLEDTLSEGIRQWWKLKPGPPPPKPAERHKDDSRGLVLPGYKYLGPFNGLDKGEPVNEADAAALEHDKAYDRQLDSGDNPYLKYNHADAEFQERLKEDTSFGGNLGRAVFQAKKRVLEPLGLVEEPVKTAPGKKRPVEHSPVEPDSSSGTGKAGQQPARKRLNFGQTGDADSVPDPQPLGQPPAAPSGLGTNTMATGSGAPMADNNEGADGVGNSSGNWHCDSTWMGDRVITTSTRTWALPTYNNHLYKQISSQSGASNDNHYFGYSTPWGYFDFNRFHCHFSPRDWQRLINNNWGFRPKRLNFKLFNIQVKEVTQNDGTTTIANNLTSTVQVFTDSEYQLPYVLGSAHQGCLPPFPADVFMVPQYGYLTLNNGSQAVGRSSFYCLEYFPSQMLRTGNNFTFSYTFEDVPFHSSYAHSQSLDRLMNPLIDQYLYYLSRTNTPSGTTTQSRLQFSQAGASDIRDQSRNWLPGPCYRQQRVSKTSADNNNSEYSWTGATKYHLNGRDSLVNPGPAMASHKDDEEKFFPQSGVLIFGKQGSEKTNVDIEKVMITDEQEVAATNPVATEAYGTVSTNLQRQNTQAATADVNTQGVLPGMVWQDRDVYLQGPIWAKIPHTDGHFHPSPLMGGFGLKHPPPQILIKNTPVPANPSTTFSAAKFASFITQYSTGQVSVEIEWELQKENSKRWNPEIQYTSNYNKSVNVDFTVDTNGVYSEPRPIGTRYLTRNL

SEQ ID NO: 23 - protein, 735 aa, synthetic construct
  source 1..735: note = Amino acid sequence of VP1 variant
MAADGYLPDWLEDTLSEGIRQWWKLKPGPPPPKPAERHKDDSRGLVLPGYKYLGPFNGLDKGEPVNEADAAALEHDKAYDRQLDSGDNPYLKYNHADAEFQERLKEDTSFGGNLGRAVFQAKKRVLEPLGLVEEPVKTAPGKKRPVEHSPVEPDSSSGTGKAGQQPARKRLNFGQTGDADSVPDPQPLGQPPAAPSGLGTNTMATGSGAPMADNNEGADGVGNSSGNWHCDSTWMGDRVITTSTRTWALPTYNNHLYKQISSQSGASNDNHYFGYSTPWGYFDFNRFHCHFSPRDWQRLINNNWGFRPKRLNFKLFNIQVKEVTQNDGTTTIANNLTSTVQVFTDSEYQLPYVLGSAHQGCLPPFPADVFMVPQYGYLTLNNGSQAVGRSSFYCLEYFPSQMLRTGNNFTFSYTFEDVPFHSSYAHSQSLDRLMNPLIDQYLYYLSRTNTPSGTTTQSRLQFSQAGASDIRDQSRNWLPGPCYRQQRVSKTSADNNNSEYSWTGATKYHLNGRDSLVNPGPAMASHKDDEEKFFPQSGVLIFGKQGSEKTNVDIEKVMITDEAEIAATNPVATEQYGTVSTNLQTGNQQAATADVNTQGVLPGMVWQDRDVYLQGPIWAKIPHTDGHFHPSPLMGGFGLKHPPPQILIKNTPVPANPSTTFSAAKFASFITQYSTGQVSVEIEWELQKENSKRWNPEIQYTSNYNKSVNVDFTVDTNGVYSEPRPIGTRYLTRNL

SEQ ID NO: 24 - protein, 735 aa, synthetic construct
  source 1..735: note = Amino acid sequence of VP1 variant
MAADGYLPDWLEDTLSEGIRQWWKLKPGPPPPKPAERHKDDSRGLVLPGYKYLGPFNGLDKGEPVNEADAAALEHDKAYDRQLDSGDNPYLKYNHADAEFQERLKEDTSFGGNLGRAVFQAKKRVLEPLGLVEEPVKTAPGKKRPVEHSPVEPDSSSGTGKAGQQPARKRLNFGQTGDADSVPDPQPLGQPPAAPSGLGTNTMATGSGAPMADNNEGADGVGNSSGNWHCDSTWMGDRVITTSTRTWALPTYNNHLYKQISSQSGASNDNHYFGYSTPWGYFDFNRFHCHFSPRDWQRLINNNWGFRPKRLNFKLFNIQVKEVTQNDGTTTIANNLTSTVQVFTDSEYQLPYVLGSAHQGCLPPFPADVFMVPQYGYLTLNNGSQAVGRSSFYCLEYFPSQMLRTGNNFTFSYTFEDVPFHSSYAHSQSLDRLMNPLIDQYLYYLSRTNTPSGTTTQSRLQFSQAGASDIRDQSRNWLPGPCYRQQRVSKTSADNNNSEYSWTGATKYHLNGRDSLVNPGPAMASHKDDEEKFFPQSGVLIFGKQGSEKTNVDIEKVMITDESEIRTTNPVATESYGEVATNLQTGTTQAATADVNTQGVLPGMVWQDRDVYLQGPIWAKIPHTDGHFHPSPLMGGFGLKHPPPQILIKNTPVPANPSTTFSAAKFASFITQYSTGQVSVEIEWELQKENSKRWNPEIQYTSNYNKSVNVDFTVDTNGVYSEPRPIGTRYLTRNL

SEQ ID NO: 25 - protein, 735 aa, synthetic construct
  source 1..735: note = Amino acid sequence of VP1 variant
MAADGYLPDWLEDTLSEGIRQWWKLKPGPPPPKPAERHKDDSRGLVLPGYKYLGPFNGLDKGEPVNEADAAALEHDKAYDRQLDSGDNPYLKYNHADAEFQERLKEDTSFGGNLGRAVFQAKKRVLEPLGLVEEPVKTAPGKKRPVEHSPVEPDSSSGTGKAGQQPARKRLNFGQTGDADSVPDPQPLGQPPAAPSGLGTNTMATGSGAPMADNNEGADGVGNSSGNWHCDSTWMGDRVITTSTRTWALPTYNNHLYKQISSQSGASNDNHYFGYSTPWGYFDFNRFHCHFSPRDWQRLINNNWGFRPKRLNFKLFNIQVKEVTQNDGTTTIANNLTSTVQVFTDSEYQLPYVLGSAHQGCLPPFPADVFMVPQYGYLTLNNGSQAVGRSSFYCLEYFPSQMLRTGNNFTFSYTFEDVPFHSSYAHSQSLDRLMNPLIDQYLYYLSRTNTPSGTTTQSRLQFSQAGASDIRDQSRNWLPGPCYRQQRVSKTSADNNNSEYSWTGATKYHLNGRDSLVNPGPAMASHKDDEEKFFPQSGVLIFGKQGSEKTNVDIEKVMITDEAEIATTNPVATEQWGSVSTNLQGGNLQAATADVNTQGVLPGMVWQDRDVYLQGPIWAKIPHTDGHFHPSPLMGGFGLKHPPPQILIKNTPVPANPSTTFSAAKFASFITQYSTGQVSVEIEWELQKENSKRWNPEIQYTSNYNKSVNVDFTVDTNGVYSEPRPIGTRYLTRNL

SEQ ID NO: 26 - protein, 735 aa, synthetic construct
  source 1..735: note = Amino acid sequence of VP1 variant
MAADGYLPDWLEDTLSEGIRQWWKLKPGPPPPKPAERHKDDSRGLVLPGYKYLGPFNGLDKGEPVNEADAAALEHDKAYDRQLDSGDNPYLKYNHADAEFQERLKEDTSFGGNLGRAVFQAKKRVLEPLGLVEEPVKTAPGKKRPVEHSPVEPDSSSGTGKAGQQPARKRLNFGQTGDADSVPDPQPLGQPPAAPSGLGTNTMATGSGAPMADNNEGADGVGNSSGNWHCDSTWMGDRVITTSTRTWALPTYNNHLYKQISSQSGASNDNHYFGYSTPWGYFDFNRFHCHFSPRDWQRLINNNWGFRPKRLNFKLFNIQVKEVTQNDGTTTIANNLTSTVQVFTDSEYQLPYVLGSAHQGCLPPFPADVFMVPQYGYLTLNNGSQAVGRSSFYCLEYFPSQMLRTGNNFTFSYTFEDVPFHSSYAHSQSLDRLMNPLIDQYLYYLSRTNTPSGTTTQSRLQFSQAGASDIRDQSRNWLPGPCYRQQRVSKTSADNNNSEYSWTGATKYHLNGRDSLVNPGPAMASHKDDEEKFFPQSGVLIFGKQGSEKTNVDIEKVMITNESEIAATNPVATEQYGVVATNLQNGTVQAATADVNTQGVLPGMVWQDRDVYLQGPIWAKIPHTDGHFHPSPLMGGFGLKHPPPQILIKNTPVPANPSTTFSAAKFASFITQYSTGQVSVEIEWELQKENSKRWNPEIQYTSNYNKSVNVDFTVDTNGVYSEPRPIGTRYLTRNL

SEQ ID NO: 27 - protein, 735 aa, synthetic construct
  source 1..735: note = Amino acid sequence of VP1 variant
MAADGYLPDWLEDTLSEGIRQWWKLKPGPPPPKPAERHKDDSRGLVLPGYKYLGPFNGLDKGEPVNEADAAALEHDKAYDRQLDSGDNPYLKYNHADAEFQERLKEDTSFGGNLGRAVFQAKKRVLEPLGLVEEPVKTAPGKKRPVEHSPVEPDSSSGTGKAGQQPARKRLNFGQTGDADSVPDPQPLGQPPAAPSGLGTNTMATGSGAPMADNNEGADGVGNSSGNWHCDSTWMGDRVITTSTRTWALPTYNNHLYKQISSQSGASNDNHYFGYSTPWGYFDFNRFHCHFSPRDWQRLINNNWGFRPKRLNFKLFNIQVKEVTQNDGTTTIANNLTSTVQVFTDSEYQLPYVLGSAHQGCLPPFPADVFMVPQYGYLTLNNGSQAVGRSSFYCLEYFPSQMLRTGNNFTFSYTFEDVPFHSSYAHSQSLDRLMNPLIDQYLYYLSRTNTPSGTTTQSRLQFSQAGASDIRDQSRNWLPGPCYRQQRVSKTSADNNNSEYSWTGATKYHLNGRDSLVNPGPAMASHKDDEEKFFPQSGVLIFGKQGSEKTNVDIEKVMITDESEIRTTNPVATEQWGEVATNLQNGNIQAATADVNTQGVLPGMVWQDRDVYLQGPIWAKIPHTDGHFHPSPLMGGFGLKHPPPQILIKNTPVPANPSTTFSAAKFASFITQYSTGQVSVEIEWELQKENSKRWNPEIQYTSNYNKSVNVDFTVDTNGVYSEPRPIGTRYLTRNL

SEQ ID NO: 28 - protein, 735 aa, synthetic construct
  source 1..735: note = Amino acid sequence of VP1 variant
MAADGYLPDWLEDTLSEGIRQWWKLKPGPPPPKPAERHKDDSRGLVLPGYKYLGPFNGLDKGEPVNEADAAALEHDKAYDRQLDSGDNPYLKYNHADAEFQERLKEDTSFGGNLGRAVFQAKKRVLEPLGLVEEPVKTAPGKKRPVEHSPVEPDSSSGTGKAGQQPARKRLNFGQTGDADSVPDPQPLGQPPAAPSGLGTNTMATGSGAPMADNNEGADGVGNSSGNWHCDSTWMGDRVITTSTRTWALPTYNNHLYKQISSQSGASNDNHYFGYSTPWGYFDFNRFHCHFSPRDWQRLINNNWGFRPKRLNFKLFNIQVKEVTQNDGTTTIANNLTSTVQVFTDSEYQLPYVLGSAHQGCLPPFPADVFMVPQYGYLTLNNGSQAVGRSSFYCLEYFPSQMLRTGNNFTFSYTFEDVPFHSSYAHSQSLDRLMNPLIDQYLYYLSRTNTPSGTTTQSRLQFSQAGASDIRDQSRNWLPGPCYRQQRVSKTSADNNNSEYSWTGATKYHLNGRDSLVNPGPAMASHKDDEEKFFPQSGVLIFGKQGSEKTNVDIEKVMITDEAEIAATNPVATEQYGCVASNIQNSNTQAATADVNTQGVLPGMVWQDRDVYLQGPIWAKIPHTDGHFHPSPLMGGFGLKHPPPQILIKNTPVPANPSTTFSAAKFASFITQYSTGQVSVEIEWELQKENSKRWNPEIQYTSNYNKSVNVDFTVDTNGVYSEPRPIGTRYLTRNL

SEQ ID NO: 29 - protein, 735 aa, synthetic construct
  source 1..735: note = Amino acid sequence of VP1 variant
MAADGYLPDWLEDTLSEGIRQWWKLKPGPPPPKPAERHKDDSRGLVLPGYKYLGPFNGLDKGEPVNEADAAALEHDKAYDRQLDSGDNPYLKYNHADAEFQERLKEDTSFGGNLGRAVFQAKKRVLEPLGLVEEPVKTAPGKKRPVEHSPVEPDSSSGTGKAGQQPARKRLNFGQTGDADSVPDPQPLGQPPAAPSGLGTNTMATGSGAPMADNNEGADGVGNSSGNWHCDSTWMGDRVITTSTRTWALPTYNNHLYKQISSQSGASNDNHYFGYSTPWGYFDFNRFHCHFSPRDWQRLINNNWGFRPKRLNFKLFNIQVKEVTQNDGTTTIANNLTSTVQVFTDSEYQLPYVLGSAHQGCLPPFPADVFMVPQYGYLTLNNGSQAVGRSSFYCLEYFPSQMLRTGNNFTFSYTFEDVPFHSSYAHSQSLDRLMNPLIDQYLYYLSRTNTPSGTTTQSRLQFSQAGASDIRDQSRNWLPGPCYRQQRVSKTSADNNNSEYSWTGATKYHLNGRDSLVNPGPAMASHKDDEEKFFPQSGVLIFGKQGSEKTNVDIEKVMITDESEIAATNPVAYEQYGSVTTNLQNGNNQAATADVNTQGVLPGMVWQDRDVYLQGPIWAKIPHTDGHFHPSPLMGGFGLKHPPPQILIKNTPVPANPSTTFSAAKFASFITQYSTGQVSVEIEWELQKENSKRWNPEIQYTSNYNKSVNVDFTVDTNGVYSEPRPIGTRYLTRNL

SEQ ID NO: 30 - protein, 735 aa, synthetic construct
  source 1..735: note = Amino acid sequence of VP1 variant
MAADGYLPDWLEDTLSEGIRQWWKLKPGPPPPKPAERHKDDSRGLVLPGYKYLGPFNGLDKGEPVNEADAAALEHDKAYDRQLDSGDNPYLKYNHADAEFQERLKEDTSFGGNLGRAVFQAKKRVLEPLGLVEEPVKTAPGKKRPVEHSPVEPDSSSGTGKAGQQPARKRLNFGQTGDADSVPDPQPLGQPPAAPSGLGTNTMATGSGAPMADNNEGADGVGNSSGNWHCDSTWMGDRVITTSTRTWALPTYNNHLYKQISSQSGASNDNHYFGYSTPWGYFDFNRFHCHFSPRDWQRLINNNWGFRPKRLNFKLFNIQVKEVTQNDGTTTIANNLTSTVQVFTDSEYQLPYVLGSAHQGCLPPFPADVFMVPQYGYLTLNNGSQAVGRSSFYCLEYFPSQMLRTGNNFTFSYTFEDVPFHSSYAHSQSLDRLMNPLIDQYLYYLSRTNTPSGTTTQSRLQFSQAGASDIRDQSRNWLPGPCYRQQRVSKTSADNNNSEYSWTGATKYHLNGRDSLVNPGPAMASHKDDEEKFFPQSGVLIFGKQGSEKTNVDIEKVMITDESEIAATNPVATEQYGCVATNLQRGYVQAATADVNTQGVLPGMVWQDRDVYLQGPIWAKIPHTDGHFHPSPLMGGFGLKHPPPQILIKNTPVPANPSTTFSAAKFASFITQYSTGQVSVEIEWELQKENSKRWNPEIQYTSNYNKSVNVDFTVDTNGVYSEPRPIGTRYLTRNL

SEQ ID NO: 31 - protein, 735 aa, synthetic construct
  source 1..735: note = Amino acid sequence of VP1 variant
MAADGYLPDWLEDTLSEGIRQWWKLKPGPPPPKPAERHKDDSRGLVLPGYKYLGPFNGLDKGEPVNEADAAALEHDKAYDRQLDSGDNPYLKYNHADAEFQERLKEDTSFGGNLGRAVFQAKKRVLEPLGLVEEPVKTAPGKKRPVEHSPVEPDSSSGTGKAGQQPARKRLNFGQTGDADSVPDPQPLGQPPAAPSGLGTNTMATGSGAPMADNNEGADGVGNSSGNWHCDSTWMGDRVITTSTRTWALPTYNNHLYKQISSQSGASNDNHYFGYSTPWGYFDFNRFHCHFSPRDWQRLINNNWGFRPKRLNFKLFNIQVKEVTQNDGTTTIANNLTSTVQVFTDSEYQLPYVLGSAHQGCLPPFPADVFMVPQYGYLTLNNGSQAVGRSSFYCLEYFPSQMLRTGNNFTFSYTFEDVPFHSSYAHSQSLDRLMNPLIDQYLYYLSRTNTPSGTTTQSRLQFSQAGASDIRDQSRNWLPGPCYRQQRVSKTSADNNNSEYSWTGATKYHLNGRDSLVNPGPAMASHKDDEEKFFPQSGVLIFGKQGSEKTNVDIEKVMITDEQEVAATNPVATEQWGEVSTNLQRGNEQAATADVNTQGVLPGMVWQDRDVYLQGPIWAKIPHTDGHFHPSPLMGGFGLKHPPPQILIKNTPVPANPSTTFSAAKFASFITQYSTGQVSVEIEWELQKENSKRWNPEIQYTSNYNKSVNVDFTVDTNGVYSEPRPIGTRYLTRNL

SEQ ID NO: 32 - protein, 598 aa, synthetic construct
  source 1..598: note = Amino acid sequence of VP2 of wild-type AAV2
TAPGKKRPVEHSPVEPDSSSGTGKAGQQPARKRLNFGQTGDADSVPDPQPLGQPPAAPSGLGTNTMATGSGAPMADNNEGADGVGNSSGNWHCDSTWMGDRVITTSTRTWALPTYNNHLYKQISSQSGASNDNHYFGYSTPWGYFDFNRFHCHFSPRDWQRLINNNWGFRPKRLNFKLFNIQVKEVTQNDGTTTIANNLTSTVQVFTDSEYQLPYVLGSAHQGCLPPFPADVFMVPQYGYLTLNNGSQAVGRSSFYCLEYFPSQMLRTGNNFTFSYTFEDVPFHSSYAHSQSLDRLMNPLIDQYLYYLSRTNTPSGTTTQSRLQFSQAGASDIRDQSRNWLPGPCYRQQRVSKTSADNNNSEYSWTGATKYHLNGRDSLVNPGPAMASHKDDEEKFFPQSGVLIFGKQGSEKTNVDIEKVMITDEEEIRTTNPVATEQYGSVSTNLQRGNRQAATADVNTQGVLPGMVWQDRDVYLQGPIWAKIPHTDGHFHPSPLMGGFGLKHPPPQILIKNTPVPANPSTTFSAAKFASFITQYSTGQVSVEIEWELQKENSKRWNPEIQYTSNYNKSVNVDFTVDTNGVYSEPRPIGTRYLTRNL

SEQ ID NO: 33 - protein, 598 aa, synthetic construct
  source 1..598: note = Amino acid sequence of VP2 variant
TAPGKKRPVEHSPVEPDSSSGTGKAGQQPARKRLNFGQTGDADSVPDPQPLGQPPAAPSGLGTNTMATGSGAPMADNNEGADGVGNSSGNWHCDSTWMGDRVITTSTRTWALPTYNNHLYKQISSQSGASNDNHYFGYSTPWGYFDFNRFHCHFSPRDWQRLINNNWGFRPKRLNFKLFNIQVKEVTQNDGTTTIANNLTSTVQVFTDSEYQLPYVLGSAHQGCLPPFPADVFMVPQYGYLTLNNGSQAVGRSSFYCLEYFPSQMLRTGNNFTFSYTFEDVPFHSSYAHSQSLDRLMNPLIDQYLYYLSRTNTPSGTTTQSRLQFSQAGASDIRDQSRNWLPGPCYRQQRVSKTSADNNNSEYSWTGATKYHLNGRDSLVNPGPAMASHKDDEEKFFPQSGVLIFGKQGSEKTNVDIEKVMITDEEEIAATNPVATESYGEVATNLQRGNVQAATADVNTQGVLPGMVWQDRDVYLQGPIWAKIPHTDGHFHPSPLMGGFGLKHPPPQILIKNTPVPANPSTTFSAAKFASFITQYSTGQVSVEIEWELQKENSKRWNPEIQYTSNYNKSVNVDFTVDTNGVYSEPRPIGTRYLTRNL

SEQ ID NO: 34 - protein, 598 aa, synthetic construct
  source 1..598: note = Amino acid sequence of VP2 variant
TAPGKKRPVEHSPVEPDSSSGTGKAGQQPARKRLNFGQTGDADSVPDPQPLGQPPAAPSGLGTNTMATGSGAPMADNNEGADGVGNSSGNWHCDSTWMGDRVITTSTRTWALPTYNNHLYKQISSQSGASNDNHYFGYSTPWGYFDFNRFHCHFSPRDWQRLINNNWGFRPKRLNFKLFNIQVKEVTQNDGTTTIANNLTSTVQVFTDSEYQLPYVLGSAHQGCLPPFPADVFMVPQYGYLTLNNGSQAVGRSSFYCLEYFPSQMLRTGNNFTFSYTFEDVPFHSSYAHSQSLDRLMNPLIDQYLYYLSRTNTPSGTTTQSRLQFSQAGASDIRDQSRNWLPGPCYRQQRVSKTSADNNNSEYSWTGATKYHLNGRDSLVNPGPAMASHKDDEEKFFPQSGVLIFGKQGSEKTNVDIEKVMITDEQEVAATNPVATESWGSVSTNLQRGNTQAATADVNTQGVLPGMVWQDRDVYLQGPIWAKIPHTDGHFHPSPLMGGFGLKHPPPQILIKNTPVPANPSTTFSAAKFASFITQYSTGQVSVEIEWELQKENSKRWNPEIQYTSNYNKSVNVDFTVDTNGVYSEPRPIGTRYLTRNL

SEQ ID NO: 35 - protein, 598 aa, synthetic construct
  source 1..598: note = Amino acid sequence of VP2 variant
TAPGKKRPVEHSPVEPDSSSGTGKAGQQPARKRLNFGQTGDADSVPDPQPLGQPPAAPSGLGTNTMATGSGAPMADNNEGADGVGNSSGNWHCDSTWMGDRVITTSTRTWALPTYNNHLYKQISSQSGASNDNHYFGYSTPWGYFDFNRFHCHFSPRDWQRLINNNWGFRPKRLNFKLFNIQVKEVTQNDGTTTIANNLTSTVQVFTDSEYQLPYVLGSAHQGCLPPFPADVFMVPQYGYLTLNNGSQAVGRSSFYCLEYFPSQMLRTGNNFTFSYTFEDVPFHSSYAHSQSLDRLMNPLIDQYLYYLSRTNTPSGTTTQSRLQFSQAGASDIRDQSRNWLPGPCYRQQRVSKTSADNNNSEYSWTGATKYHLNGRDSLVNPGPAMASHKDDEEKFFPQSGVLIFGKQGSEKTNVDIEKVMITDESEIRTTNPIATEQWGSVSTNLQNGNRQAATADVNTQGVLPGMVWQDRDVYLQGPIWAKIPHTDGHFHPSPLMGGFGLKHPPPQILIKNTPVPANPSTTFSAAKFASFITQYSTGQVSVEIEWELQKENSKRWNPEIQYTSNYNKSVNVDFTVDTNGVYSEPRPIGTRYLTRNL

SEQ ID NO: 36 - protein, 598 aa, synthetic construct
  source 1..598: note = Amino acid sequence of VP2 variant
TAPGKKRPVEHSPVEPDSSSGTGKAGQQPARKRLNFGQTGDADSVPDPQPLGQPPAAPSGLGTNTMATGSGAPMADNNEGADGVGNSSGNWHCDSTWMGDRVITTSTRTWALPTYNNHLYKQISSQSGASNDNHYFGYSTPWGYFDFNRFHCHFSPRDWQRLINNNWGFRPKRLNFKLFNIQVKEVTQNDGTTTIANNLTSTVQVFTDSEYQLPYVLGSAHQGCLPPFPADVFMVPQYGYLTLNNGSQAVGRSSFYCLEYFPSQMLRTGNNFTFSYTFEDVPFHSSYAHSQSLDRLMNPLIDQYLYYLSRTNTPSGTTTQSRLQFSQAGASDIRDQSRNWLPGPCYRQQRVSKTSADNNNSEYSWTGATKYHLNGRDSLVNPGPAMASHKDDEEKFFPQSGVLIFGKQGSEKTNVDIEKVMITDEEEIATTNPVATEQWGSVSTNLQRGATQAATADVNTQGVLPGMVWQDRDVYLQGPIWAKIPHTDGHFHPSPLMGGFGLKHPPPQILIKNTPVPANPSTTFSAAKFASFITQYSTGQVSVEIEWELQKENSKRWNPEIQYTSNYNKSVNVDFTVDTNGVYSEPRPIGTRYLTRNL

SEQ ID NO: 37 - protein, 598 aa, synthetic construct
  source 1..598: note = Amino acid sequence of VP2 variant
TAPGKKRPVEHSPVEPDSSSGTGKAGQQPARKRLNFGQTGDADSVPDPQPLGQPPAAPSGLGTNTMATGSGAPMADNNEGADGVGNSSGNWHCDSTWMGDRVITTSTRTWALPTYNNHLYKQISSQSGASNDNHYFGYSTPWGYFDFNRFHCHFSPRDWQRLINNNWGFRPKRLNFKLFNIQVKEVTQNDGTTTIANNLTSTVQVFTDSEYQLPYVLGSAHQGCLPPFPADVFMVPQYGYLTLNNGSQAVGRSSFYCLEYFPSQMLRTGNNFTFSYTFEDVPFHSSYAHSQSLDRLMNPLIDQYLYYLSRTNTPSGTTTQSRLQFSQAGASDIRDQSRNWLPGPCYRQQRVSKTSADNNNSEYSWTGATKYHLNGRDSLVNPGPAMASHKDDEEKFFPQSGVLIFGKQGSEKTNVDIEKVMITDESEIATTNPVATESYGEVSTNLQRNPVQAATADVNTQGVLPGMVWQDRDVYLQGPIWAKIPHTDGHFHPSPLMGGFGLKHPPPQILIKNTPVPANPSTTFSAAKFASFITQYSTGQVSVEIEWELQKENSKRWNPEIQYTSNYNKSVNVDFTVDTNGVYSEPRPIGTRYLTRNL

SEQ ID NO: 38 - protein, 598 aa, synthetic construct
  source 1..598: note = Amino acid sequence of VP2 variant
TAPGKKRPVEHSPVEPDSSSGTGKAGQQPARKRLNFGQTGDADSVPDPQPLGQPPAAPSGLGTNTMATGSGAPMADNNEGADGVGNSSGNWHCDSTWMGDRVITTSTRTWALPTYNNHLYKQISSQSGASNDNHYFGYSTPWGYFDFNRFHCHFSPRDWQRLINNNWGFRPKRLNFKLFNIQVKEVTQNDGTTTIANNLTSTVQVFTDSEYQLPYVLGSAHQGCLPPFPADVFMVPQYGYLTLNNGSQAVGRSSFYCLEYFPSQMLRTGNNFTFSYTFEDVPFHSSYAHSQSLDRLMNPLIDQYLYYLSRTNTPSGTTTQSRLQFSQAGASDIRDQSRNWLPGPCYRQQRVSKTSADNNNSEYSWTGATKYHLNGRDSLVNPGPAMASHKDDEEKFFPQSGVLIFGKQGSEKTNVDIEKVMITDEEEIRTTNPVAYEQYGVVATNLQNSNAQAATADVNTQGVLPGMVWQDRDVYLQGPIWAKIPHTDGHFHPSPLMGGFGLKHPPPQILIKNTPVPANPSTTFSAAKFASFITQYSTGQVSVEIEWELQKENSKRWNPEIQYTSNYNKSVNVDFTVDTNGVYSEPRPIGTRYLTRNL

SEQ ID NO: 39 - protein, 598 aa, synthetic construct
  source 1..598: note = Amino acid sequence of VP2 variant
TAPGKKRPVEHSPVEPDSSSGTGKAGQQPARKRLNFGQTGDADSVPDPQPLGQPPAAPSGLGTNTMATGSGAPMADNNEGADGVGNSSGNWHCDSTWMGDRVITTSTRTWALPTYNNHLYKQISSQSGASNDNHYFGYSTPWGYFDFNRFHCHFSPRDWQRLINNNWGFRPKRLNFKLFNIQVKEVTQNDGTTTIANNLTSTVQVFTDSEYQLPYVLGSAHQGCLPPFPADVFMVPQYGYLTLNNGSQAVGRSSFYCLEYFPSQMLRTGNNFTFSYTFEDVPFHSSYAHSQSLDRLMNPLIDQYLYYLSRTNTPSGTTTQSRLQFSQAGASDIRDQSRNWLPGPCYRQQRVSKTSADNNNSEYSWTGATKYHLNGRDSLVNPGPAMASHKDDEEKFFPQSGVLIFGKQGSEKTNVDIEKVMITDEAEIATTNPVAAEQYGEVSTNLQNGNRQAATADVNTQGVLPGMVWQDRDVYLQGPIWAKIPHTDGHFHPSPLMGGFGLKHPPPQILIKNTPVPANPSTTFSAAKFASFITQYSTGQVSVEIEWELQKENSKRWNPEIQYTSNYNKSVNVDFTVDTNGVYSEPRPIGTRYLTRNL

SEQ ID NO: 40 - protein, 598 aa, synthetic construct
  source 1..598: note = Amino acid sequence of VP2 variant
TAPGKKRPVEHSPVEPDSSSGTGKAGQQPARKRLNFGQTGDADSVPDPQPLGQPPAAPSGLGTNTMATGSGAPMADNNEGADGVGNSSGNWHCDSTWMGDRVITTSTRTWALPTYNNHLYKQISSQSGASNDNHYFGYSTPWGYFDFNRFHCHFSPRDWQRLINNNWGFRPKRLNFKLFNIQVKEVTQNDGTTTIANNLTSTVQVFTDSEYQLPYVLGSAHQGCLPPFPADVFMVPQYGYLTLNNGSQAVGRSSFYCLEYFPSQMLRTGNNFTFSYTFEDVPFHSSYAHSQSLDRLMNPLIDQYLYYLSRTNTPSGTTTQSRLQFSQAGASDIRDQSRNWLPGPCYRQQRVSKTSADNNNSEYSWTGATKYHLNGRDSLVNPGPAMASHKDDEEKFFPQSGVLIFGKQGSEKTNVDIEKVMITDEQEVAATNPVATEHYGQVATNLQTGNRQAATADVNTQGVLPGMVWQDRDVYLQGPIWAKIPHTDGHFHPSPLMGGFGLKHPPPQILIKNTPVPANPSTTFSAAKFASFITQYSTGQVSVEIEWELQKENSKRWNPEIQYTSNYNKSVNVDFTVDTNGVYSEPRPIGTRYLTRNL

SEQ ID NO: 41 - protein, 598 aa, synthetic construct
  source 1..598: note = Amino acid sequence of VP2 variant
TAPGKKRPVEHSPVEPDSSSGTGKAGQQPARKRLNFGQTGDADSVPDPQPLGQPPAAPSGLGTNTMATGSGAPMADNNEGADGVGNSSGNWHCDSTWMGDRVITTSTRTWALPTYNNHLYKQISSQSGASNDNHYFGYSTPWGYFDFNRFHCHFSPRDWQRLINNNWGFRPKRLNFKLFNIQVKEVTQNDGTTTIANNLTSTVQVFTDSEYQLPYVLGSAHQGCLPPFPADVFMVPQYGYLTLNNGSQAVGRSSFYCLEYFPSQMLRTGNNFTFSYTFEDVPFHSSYAHSQSLDRLMNPLIDQYLYYLSRTNTPSGTTTQSRLQFSQAGASDIRDQSRNWLPGPCYRQQRVSKTSADNNNSEYSWTGATKYHLNGRDSLVNPGPAMASHKDDEEKFFPQSGVLIFGKQGSEKTNVDIEKVMITDEEEINTTNPVYTEQYGSVSTNLQRGNIQAATADVNTQGVLPGMVWQDRDVYLQGPIWAKIPHTDGHFHPSPLMGGFGLKHPPPQILIKNTPVPANPSTTFSAAKFASFITQYSTGQVSVEIEWELQKENSKRWNPEIQYTSNYNKSVNVDFTVDTNGVYSEPRPIGTRYLTRNL

SEQ ID NO: 42 - protein, 598 aa, synthetic construct
  source 1..598: note = Amino acid sequence of VP2 variant
TAPGKKRPVEHSPVEPDSSSGTGKAGQQPARKRLNFGQTGDADSVPDPQPLGQPPAAPSGLGTNTMATGSGAPMADNNEGADGVGNSSGNWHCDSTWMGDRVITTSTRTWALPTYNNHLYKQISSQSGASNDNHYFGYSTPWGYFDFNRFHCHFSPRDWQRLINNNWGFRPKRLNFKLFNIQVKEVTQNDGTTTIANNLTSTVQVFTDSEYQLPYVLGSAHQGCLPPFPADVFMVPQYGYLTLNNGSQAVGRSSFYCLEYFPSQMLRTGNNFTFSYTFEDVPFHSSYAHSQSLDRLMNPLIDQYLYYLSRTNTPSGTTTQSRLQFSQAGASDIRDQSRNWLPGPCYRQQRVSKTSADNNNSEYSWTGATKYHLNGRDSLVNPGPAMASHKDDEEKFFPQSGVLIFGKQGSEKTNVDIEKVMITDEQEVAATNPVADEQYGVVATNLQRGNVQAATADVNTQGVLPGMVWQDRDVYLQGPIWAKIPHTDGHFHPSPLMGGFGLKHPPPQILIKNTPVPANPSTTFSAAKFASFITQYSTGQVSVEIEWELQKENSKRWNPEIQYTSNYNKSVNVDFTVDTNGVYSEPRPIGTRYLTRNL

SEQ ID NO: 43 - protein, 598 aa, synthetic construct
  source 1..598: note = Amino acid sequence of VP2 variant
TAPGKKRPVEHSPVEPDSSSGTGKAGQQPARKRLNFGQTGDADSVPDPQPLGQPPAAPSGLGTNTMATGSGAPMADNNEGADGVGNSSGNWHCDSTWMGDRVITTSTRTWALPTYNNHLYKQISSQSGASNDNHYFGYSTPWGYFDFNRFHCHFSPRDWQRLINNNWGFRPKRLNFKLFNIQVKEVTQNDGTTTIANNLTSTVQVFTDSEYQLPYVLGSAHQGCLPPFPADVFMVPQYGYLTLNNGSQAVGRSSFYCLEYFPSQMLRTGNNFTFSYTFEDVPFHSSYAHSQSLDRLMNPLIDQYLYYLSRTNTPSGTTTQSRLQFSQAGASDIRDQSRNWLPGPCYRQQRVSKTSADNNNSEYSWTGATKYHLNGRDSLVNPGPAMASHKDDEEKFFPQSGVLIFGKQGSEKTNVDIEKVMITDESEIAATNPVATEQWGSVATNRQRGETQAATADVNTQGVLPGMVWQDRDVYLQGPIWAKIPHTDGHFHPSPLMGGFGLKHPPPQILIKNTPVPANPSTTFSAAKFASFITQYSTGQVSVEIEWELQKENSKRWNPEIQYTSNYNKSVNVDFTVDTNGVYSEPRPIGTRYLTRNL

SEQ ID NO: 44 - protein, 598 aa, synthetic construct
  source 1..598: note = Amino acid sequence of VP2 variant
TAPGKKRPVEHSPVEPDSSSGTGKAGQQPARKRLNFGQTGDADSVPDPQPLGQPPAAPSGLGTNTMATGSGAPMADNNEGADGVGNSSGNWHCDSTWMGDRVITTSTRTWALPTYNNHLYKQISSQSGASNDNHYFGYSTPWGYFDFNRFHCHFSPRDWQRLINNNWGFRPKRLNFKLFNIQVKEVTQNDGTTTIANNLTSTVQVFTDSEYQLPYVLGSAHQGCLPPFPADVFMVPQYGYLTLNNGSQAVGRSSFYCLEYFPSQMLRTGNNFTFSYTFEDVPFHSSYAHSQSLDRLMNPLIDQYLYYLSRTNTPSGTTTQSRLQFSQAGASDIRDQSRNWLPGPCYRQQRVSKTSADNNNSEYSWTGATKYHLNGRDSLVNPGPAMASHKDDEEKFFPQSGVLIFGKQGSEKTNVDIEKVMITDEQEVAATNPVATEQWGEVSTNLQRSTTQAATADVNTQGVLPGMVWQDRDVYLQGPIWAKIPHTDGHFHPSPLMGGFGLKHPPPQILIKNTPVPANPSTTFSAAKFASFITQYSTGQVSVEIEWELQKENSKRWNPEIQYTSNYNKSVNVDFTVDTNGVYSEPRPIGTRYLTRNL

SEQ ID NO: 45 - protein, 598 aa, synthetic construct
  source 1..598: note = Amino acid sequence of VP2 variant
TAPGKKRPVEHSPVEPDSSSGTGKAGQQPARKRLNFGQTGDADSVPDPQPLGQPPAAPSGLGTNTMATGSGAPMADNNEGADGVGNSSGNWHCDSTWMGDRVITTSTRTWALPTYNNHLYKQISSQSGASNDNHYFGYSTPWGYFDFNRFHCHFSPRDWQRLINNNWGFRPKRLNFKLFNIQVKEVTQNDGTTTIANNLTSTVQVFTDSEYQLPYVLGSAHQGCLPPFPADVFMVPQYGYLTLNNGSQAVGRSSFYCLEYFPSQMLRTGNNFTFSYTFEDVPFHSSYAHSQSLDRLMNPLIDQYLYYLSRTNTPSGTTTQSRLQFSQAGASDIRDQSRNWLPGPCYRQQRVSKTSADNNNSEYSWTGATKYHLNGRDSLVNPGPAMASHKDDEEKFFPQSGVLIFGKQGSEKTNVDIEKVMITQESEIAATNPVATEQWGVVATNLQNGTRQAATADVNTQGVLPGMVWQDRDVYLQGPIWAKIPHTDGHFHPSPLMGGFGLKHPPPQILIKNTPVPANPSTTFSAAKFASFITQYSTGQVSVEIEWELQKENSKRWNPEIQYTSNYNKSVNVDFTVDTNGVYSEPRPIGTRYLTRNL

SEQ ID NO: 46 - protein, 598 aa, synthetic construct
  source 1..598: note = Amino acid sequence of VP2 variant
TAPGKKRPVEHSPVEPDSSSGTGKAGQQPARKRLNFGQTGDADSVPDPQPLGQPPAAPSGLGTNTMATGSGAPMADNNEGADGVGNSSGNWHCDSTWMGDRVITTSTRTWALPTYNNHLYKQISSQSGASNDNHYFGYSTPWGYFDFNRFHCHFSPRDWQRLINNNWGFRPKRLNFKLFNIQVKEVTQNDGTTTIANNLTSTVQVFTDSEYQLPYVLGSAHQGCLPPFPADVFMVPQYGYLTLNNGSQAVGRSSFYCLEYFPSQMLRTGNNFTFSYTFEDVPFHSSYAHSQSLDRLMNPLIDQYLYYLSRTNTPSGTTTQSRLQFSQAGASDIRDQSRNWLPGPCYRQQRVSKTSADNNNSEYSWTGATKYHLNGRDSLVNPGPAMASHKDDEEKFFPQSGVLIFGKQGSEKTNVDIEKVMITDESEVAATNPVATEQWGEVSTNNQRGTTQAATADVNTQGVLPGMVWQDRDVYLQGPIWAKIPHTDGHFHPSPLMGGFGLKHPPPQILIKNTPVPANPSTTFSAAKFASFITQYSTGQVSVEIEWELQKENSKRWNPEIQYTSNYNKSVNVDFTVDTNGVYSEPRPIGTRYLTRNL

SEQ ID NO: 47 - protein, 598 aa, synthetic construct
  source 1..598: note = Amino acid sequence of VP2 variant
TAPGKKRPVEHSPVEPDSSSGTGKAGQQPARKRLNFGQTGDADSVPDPQPLGQPPAAPSGLGTNTMATGSGAPMADNNEGADGVGNSSGNWHCDSTWMGDRVITTSTRTWALPTYNNHLYKQISSQSGASNDNHYFGYSTPWGYFDFNRFHCHFSPRDWQRLINNNWGFRPKRLNFKLFNIQVKEVTQNDGTTTIANNLTSTVQVFTDSEYQLPYVLGSAHQGCLPPFPADVFMVPQYGYLTLNNGSQAVGRSSFYCLEYFPSQMLRTGNNFTFSYTFEDVPFHSSYAHSQSLDRLMNPLIDQYLYYLSRTNTPSGTTTQSRLQFSQAGASDIRDQSRNWLPGPCYRQQRVSKTSADNNNSEYSWTGATKYHLNGRDSLVNPGPAMASHKDDEEKFFPQSGVLIFGKQGSEKTNVDIEKVMITDEEEIRTTNPVATEQYGSVSTNIQHGNRQAATADVNTQGVLPGMVWQDRDVYLQGPIWAKIPHTDGHFHPSPLMGGFGLKHPPPQILIKNTPVPANPSTTFSAAKFASFITQYSTGQVSVEIEWELQKENSKRWNPEIQYTSNYNKSVNVDFTVDTNGVYSEPRPIGTRYLTRNL

SEQ ID NO: 48 - protein, 598 aa, synthetic construct
  source 1..598: note = Amino acid sequence of VP2 variant
TAPGKKRPVEHSPVEPDSSSGTGKAGQQPARKRLNFGQTGDADSVPDPQPLGQPPAAPSGLGTNTMATGSGAPMADNNEGADGVGNSSGNWHCDSTWMGDRVITTSTRTWALPTYNNHLYKQISSQSGASNDNHYFGYSTPWGYFDFNRFHCHFSPRDWQRLINNNWGFRPKRLNFKLFNIQVKEVTQNDGTTTIANNLTSTVQVFTDSEYQLPYVLGSAHQGCLPPFPADVFMVPQYGYLTLNNGSQAVGRSSFYCLEYFPSQMLRTGNNFTFSYTFEDVPFHSSYAHSQSLDRLMNPLIDQYLYYLSRTNTPSGTTTQSRLQFSQAGASDIRDQSRNWLPGPCYRQQRVSKTSADNNNSEYSWTGATKYHLNGRDSLVNPGPAMASHKDDEEKFFPQSGVLIFGKQGSEKTNVDIEKVMITDEEEIRTTNPVATEQYGSVSTWLQRGNRQAATADVNTQGVLPGMVWQDRDVYLQGPIWAKIPHTDGHFHPSPLMGGFGLKHPPPQILIKNTPVPANPSTTFSAAKFASFITQYSTGQVSVEIEWELQKENSKRWNPEIQYTSNYNKSVNVDFTVDTNGVYSEPRPIGTRYLTRNL

SEQ ID NO: 49 - protein, 598 aa, synthetic construct
  source 1..598: note = Amino acid sequence of VP2 variant
TAPGKKRPVEHSPVEPDSSSGTGKAGQQPARKRLNFGQTGDADSVPDPQPLGQPPAAPSGLGTNTMATGSGAPMADNNEGADGVGNSSGNWHCDSTWMGDRVITTSTRTWALPTYNNHLYKQISSQSGASNDNHYFGYSTPWGYFDFNRFHCHFSPRDWQRLINNNWGFRPKRLNFKLFNIQVKEVTQNDGTTTIANNLTSTVQVFTDSEYQLPYVLGSAHQGCLPPFPADVFMVPQYGYLTLNNGSQAVGRSSFYCLEYFPSQMLRTGNNFTFSYTFEDVPFHSSYAHSQSLDRLMNPLIDQYLYYLSRTNTPSGTTTQSRLQFSQAGASDIRDQSRNWLPGPCYRQQRVSKTSADNNNSEYSWTGATKYHLNGRDSLVNPGPAMASHKDDEEKFFPQSGVLIFGKQGSEKTNVDIEKVMITDEQEIAATNPVATEQYGEVSTNLQNQNRQAATADVNTQGVLPGMVWQDRDVYLQGPIWAKIPHTDGHFHPSPLMGGFGLKHPPPQILIKNTPVPANPSTTFSAAKFASFITQYSTGQVSVEIEWELQKENSKRWNPEIQYTSNYNKSVNVDFTVDTNGVYSEPRPIGTRYLTRNL

SEQ ID NO: 50 - protein, 598 aa, synthetic construct
  source 1..598: note = Amino acid sequence of VP2 variant
TAPGKKRPVEHSPVEPDSSSGTGKAGQQPARKRLNFGQTGDADSVPDPQPLGQPPAAPSGLGTNTMATGSGAPMADNNEGADGVGNSSGNWHCDSTWMGDRVITTSTRTWALPTYNNHLYKQISSQSGASNDNHYFGYSTPWGYFDFNRFHCHFSPRDWQRLINNNWGFRPKRLNFKLFNIQVKEVTQNDGTTTIANNLTSTVQVFTDSEYQLPYVLGSAHQGCLPPFPADVFMVPQYGYLTLNNGSQAVGRSSFYCLEYFPSQMLRTGNNFTFSYTFEDVPFHSSYAHSQSLDRLMNPLIDQYLYYLSRTNTPSGTTTQSRLQFSQAGASDIRDQSRNWLPGPCYRQQRVSKTSADNNNSEYSWTGATKYHLNGRDSLVNPGPAMASHKDDEEKFFPQSGVLIFGKQGSEKTNVDIEKVMITQESEIAATNPVATEQWGEVATNLQRGTTQAATADVNTQGVLPGMVWQDRDVYLQGPIWAKIPHTDGHFHPSPLMGGFGLKHPPPQILIKNTPVPANPSTTFSAAKFASFITQYSTGQVSVEIEWELQKENSKRWNPEIQYTSNYNKSVNVDFTVDTNGVYSEPRPIGTRYLTRNL

SEQ ID NO: 51 - protein, 598 aa, synthetic construct
  source 1..598: note = Amino acid sequence of VP2 variant
TAPGKKRPVEHSPVEPDSSSGTGKAGQQPARKRLNFGQTGDADSVPDPQPLGQPPAAPSGLGTNTMATGSGAPMADNNEGADGVGNSSGNWHCDSTWMGDRVITTSTRTWALPTYNNHLYKQISSQSGASNDNHYFGYSTPWGYFDFNRFHCHFSPRDWQRLINNNWGFRPKRLNFKLFNIQVKEVTQNDGTTTIANNLTSTVQVFTDSEYQLPYVLGSAHQGCLPPFPADVFMVPQYGYLTLNNGSQAVGRSSFYCLEYFPSQMLRTGNNFTFSYTFEDVPFHSSYAHSQSLDRLMNPLIDQYLYYLSRTNTPSGTTTQSRLQFSQAGASDIRDQSRNWLPGPCYRQQRVSKTSADNNNSEYSWTGATKYHLNGRDSLVNPGPAMASHKDDEEKFFPQSGVLIFGKQGSEKTNVDIEKVMITDEWEIRTTNPVATEQYGSVSTNLQRLNRQAATADVNTQGVLPGMVWQDRDVYLQGPIWAKIPHTDGHFHPSPLMGGFGLKHPPPQILIKNTPVPANPSTTFSAAKFASFITQYSTGQVSVEIEWELQKENSKRWNPEIQYTSNYNKSVNVDFTVDTNGVYSEPRPIGTRYLTRNL

SEQ ID NO: 52 - protein, 598 aa, synthetic construct
  source 1..598: note = Amino acid sequence of VP2 variant
TAPGKKRPVEHSPVEPDSSSGTGKAGQQPARKRLNFGQTGDADSVPDPQPLGQPPAAPSGLGTNTMATGSGAPMADNNEGADGVGNSSGNWHCDSTWMGDRVITTSTRTWALPTYNNHLYKQISSQSGASNDNHYFGYSTPWGYFDFNRFHCHFSPRDWQRLINNNWGFRPKRLNFKLFNIQVKEVTQNDGTTTIANNLTSTVQVFTDSEYQLPYVLGSAHQGCLPPFPADVFMVPQYGYLTLNNGSQAVGRSSFYCLEYFPSQMLRTGNNFTFSYTFEDVPFHSSYAHSQSLDRLMNPLIDQYLYYLSRTNTPSGTTTQSRLQFSQAGASDIRDQSRNWLPGPCYRQQRVSKTSADNNNSEYSWTGATKYHLNGRDSLVNPGPAMASHKDDEEKFFPQSGVLIFGKQGSEKTNVDIEKVMITDEAEIAATNPVATEQWGEVSTNTQNGARQAATADVNTQGVLPGMVWQDRDVYLQGPIWAKIPHTDGHFHPSPLMGGFGLKHPPPQILIKNTPVPANPSTTFSAAKFASFITQYSTGQVSVEIEWELQKENSKRWNPEIQYTSNYNKSVNVDFTVDTNGVYSEPRPIGTRYLTRNL

SEQ ID NO: 53 - protein, 598 aa, synthetic construct
  source 1..598: note = Amino acid sequence of VP2 variant
TAPGKKRPVEHSPVEPDSSSGTGKAGQQPARKRLNFGQTGDADSVPDPQPLGQPPAAPSGLGTNTMATGSGAPMADNNEGADGVGNSSGNWHCDSTWMGDRVITTSTRTWALPTYNNHLYKQISSQSGASNDNHYFGYSTPWGYFDFNRFHCHFSPRDWQRLINNNWGFRPKRLNFKLFNIQVKEVTQNDGTTTIANNLTSTVQVFTDSEYQLPYVLGSAHQGCLPPFPADVFMVPQYGYLTLNNGSQAVGRSSFYCLEYFPSQMLRTGNNFTFSYTFEDVPFHSSYAHSQSLDRLMNPLIDQYLYYLSRTNTPSGTTTQSRLQFSQAGASDIRDQSRNWLPGPCYRQQRVSKTSADNNNSEYSWTGATKYHLNGRDSLVNPGPAMASHKDDEEKFFPQSGVLIFGKQGSEKTNVDIEKVMITDEQEVAATNPVATEAYGTVSTNLQRQNTQAATADVNTQGVLPGMVWQDRDVYLQGPIWAKIPHTDGHFHPSPLMGGFGLKHPPPQILIKNTPVPANPSTTFSAAKFASFITQYSTGQVSVEIEWELQKENSKRWNPEIQYTSNYNKSVNVDFTVDTNGVYSEPRPIGTRYLTRNL

SEQ ID NO: 54 - protein, 598 aa, synthetic construct
  source 1..598: note = Amino acid sequence of VP2 variant
TAPGKKRPVEHSPVEPDSSSGTGKAGQQPARKRLNFGQTGDADSVPDPQPLGQPPAAPSGLGTNTMATGSGAPMADNNEGADGVGNSSGNWHCDSTWMGDRVITTSTRTWALPTYNNHLYKQISSQSGASNDNHYFGYSTPWGYFDFNRFHCHFSPRDWQRLINNNWGFRPKRLNFKLFNIQVKEVTQNDGTTTIANNLTSTVQVFTDSEYQLPYVLGSAHQGCLPPFPADVFMVPQYGYLTLNNGSQAVGRSSFYCLEYFPSQMLRTGNNFTFSYTFEDVPFHSSYAHSQSLDRLMNPLIDQYLYYLSRTNTPSGTTTQSRLQFSQAGASDIRDQSRNWLPGPCYRQQRVSKTSADNNNSEYSWTGATKYHLNGRDSLVNPGPAMASHKDDEEKFFPQSGVLIFGKQGSEKTNVDIEKVMITDEAEIAATNPVATEQYGTVSTNLQTGNQQAATADVNTQGVLPGMVWQDRDVYLQGPIWAKIPHTDGHFHPSPLMGGFGLKHPPPQILIKNTPVPANPSTTFSAAKFASFITQYSTGQVSVEIEWELQKENSKRWNPEIQYTSNYNKSVNVDFTVDTNGVYSEPRPIGTRYLTRNL

SEQ ID NO: 55 - protein, 598 aa, synthetic construct
  source 1..598: note = Amino acid sequence of VP2 variant
TAPGKKRPVEHSPVEPDSSSGTGKAGQQPARKRLNFGQTGDADSVPDPQPLGQPPAAPSGLGTNTMATGSGAPMADNNEGADGVGNSSGNWHCDSTWMGDRVITTSTRTWALPTYNNHLYKQISSQSGASNDNHYFGYSTPWGYFDFNRFHCHFSPRDWQRLINNNWGFRPKRLNFKLFNIQVKEVTQNDGTTTIANNLTSTVQVFTDSEYQLPYVLGSAHQGCLPPFPADVFMVPQYGYLTLNNGSQAVGRSSFYCLEYFPSQMLRTGNNFTFSYTFEDVPFHSSYAHSQSLDRLMNPLIDQYLYYLSRTNTPSGTTTQSRLQFSQAGASDIRDQSRNWLPGPCYRQQRVSKTSADNNNSEYSWTGATKYHLNGRDSLVNPGPAMASHKDDEEKFFPQSGVLIFGKQGSEKTNVDIEKVMITDESEIRTTNPVATESYGEVATNLQTGTTQAATADVNTQGVLPGMVWQDRDVYLQGPIWAKIPHTDGHFHPSPLMGGFGLKHPPPQILIKNTPVPANPSTTFSAAKFASFITQYSTGQVSVEIEWELQKENSKRWNPEIQYTSNYNKSVNVDFTVDTNGVYSEPRPIGTRYLTRNL

SEQ ID NO: 56 - protein, 598 aa, synthetic construct
  source 1..598: note = Amino acid sequence of VP2 variant
TAPGKKRPVEHSPVEPDSSSGTGKAGQQPARKRLNFGQTGDADSVPDPQPLGQPPAAPSGLGTNTMATGSGAPMADNNEGADGVGNSSGNWHCDSTWMGDRVITTSTRTWALPTYNNHLYKQISSQSGASNDNHYFGYSTPWGYFDFNRFHCHFSPRDWQRLINNNWGFRPKRLNFKLFNIQVKEVTQNDGTTTIANNLTSTVQVFTDSEYQLPYVLGSAHQGCLPPFPADVFMVPQYGYLTLNNGSQAVGRSSFYCLEYFPSQMLRTGNNFTFSYTFEDVPFHSSYAHSQSLDRLMNPLIDQYLYYLSRTNTPSGTTTQSRLQFSQAGASDIRDQSRNWLPGPCYRQQRVSKTSADNNNSEYSWTGATKYHLNGRDSLVNPGPAMASHKDDEEKFFPQSGVLIFGKQGSEKTNVDIEKVMITDEAEIATTNPVATEQWGSVSTNLQGGNLQAATADVNTQGVLPGMVWQDRDVYLQGPIWAKIPHTDGHFHPSPLMGGFGLKHPPPQILIKNTPVPANPSTTFSAAKFASFITQYSTGQVSVEIEWELQKENSKRWNPEIQYTSNYNKSVNVDFTVDTNGVYSEPRPIGTRYLTRNL

SEQ ID NO: 57 - protein, 598 aa, synthetic construct
  source 1..598: note = Amino acid sequence of VP2 variant
TAPGKKRPVEHSPVEPDSSSGTGKAGQQPARKRLNFGQTGDADSVPDPQPLGQPPAAPSGLGTNTMATGSGAPMADNNEGADGVGNSSGNWHCDSTWMGDRVITTSTRTWALPTYNNHLYKQISSQSGASNDNHYFGYSTPWGYFDFNRFHCHFSPRDWQRLINNNWGFRPKRLNFKLFNIQVKEVTQNDGTTTIANNLTSTVQVFTDSEYQLPYVLGSAHQGCLPPFPADVFMVPQYGYLTLNNGSQAVGRSSFYCLEYFPSQMLRTGNNFTFSYTFEDVPFHSSYAHSQSLDRLMNPLIDQYLYYLSRTNTPSGTTTQSRLQFSQAGASDIRDQSRNWLPGPCYRQQRVSKTSADNNNSEYSWTGATKYHLNGRDSLVNPGPAMASHKDDEEKFFPQSGVLIFGKQGSEKTNVDIEKVMITNESEIAATNPVATEQYGVVATNLQNGTVQAATADVNTQGVLPGMVWQDRDVYLQGPIWAKIPHTDGHFHPSPLMGGFGLKHPPPQILIKNTPVPANPSTTFSAAKFASFITQYSTGQVSVEIEWELQKENSKRWNPEIQYTSNYNKSVNVDFTVDTNGVYSEPRPIGTRYLTRNL

SEQ ID NO: 58 - protein, 598 aa, synthetic construct
  source 1..598: note = Amino acid sequence of VP2 variant
TAPGKKRPVEHSPVEPDSSSGTGKAGQQPARKRLNFGQTGDADSVPDPQPLGQPPAAPSGLGTNTMATGSGAPMADNNEGADGVGNSSGNWHCDSTWMGDRVITTSTRTWALPTYNNHLYKQISSQSGASNDNHYFGYSTPWGYFDFNRFHCHFSPRDWQRLINNNWGFRPKRLNFKLFNIQVKEVTQNDGTTTIANNLTSTVQVFTDSEYQLPYVLGSAHQGCLPPFPADVFMVPQYGYLTLNNGSQAVGRSSFYCLEYFPSQMLRTGNNFTFSYTFEDVPFHSSYAHSQSLDRLMNPLIDQYLYYLSRTNTPSGTTTQSRLQFSQAGASDIRDQSRNWLPGPCYRQQRVSKTSADNNNSEYSWTGATKYHLNGRDSLVNPGPAMASHKDDEEKFFPQSGVLIFGKQGSEKTNVDIEKVMITDESEIRTTNPVATEQWGEVATNLQNGNIQAATADVNTQGVLPGMVWQDRDVYLQGPIWAKIPHTDGHFHPSPLMGGFGLKHPPPQILIKNTPVPANPSTTFSAAKFASFITQYSTGQVSVEIEWELQKENSKRWNPEIQYTSNYNKSVNVDFTVDTNGVYSEPRPIGTRYLTRNL

SEQ ID NO: 59 - protein, 598 aa, synthetic construct
  source 1..598: note = Amino acid sequence of VP2 variant
TAPGKKRPVEHSPVEPDSSSGTGKAGQQPARKRLNFGQTGDADSVPDPQPLGQPPAAPSGLGTNTMATGSGAPMADNNEGADGVGNSSGNWHCDSTWMGDRVITTSTRTWALPTYNNHLYKQISSQSGASNDNHYFGYSTPWGYFDFNRFHCHFSPRDWQRLINNNWGFRPKRLNFKLFNIQVKEVTQNDGTTTIANNLTSTVQVFTDSEYQLPYVLGSAHQGCLPPFPADVFMVPQYGYLTLNNGSQAVGRSSFYCLEYFPSQMLRTGNNFTFSYTFEDVPFHSSYAHSQSLDRLMNPLIDQYLYYLSRTNTPSGTTTQSRLQFSQAGASDIRDQSRNWLPGPCYRQQRVSKTSADNNNSEYSWTGATKYHLNGRDSLVNPGPAMASHKDDEEKFFPQSGVLIFGKQGSEKTNVDIEKVMITDEAEIAATNPVATEQYGCVASNIQNSNTQAATADVNTQGVLPGMVWQDRDVYLQGPIWAKIPHTDGHFHPSPLMGGFGLKHPPPQILIKNTPVPANPSTTFSAAKFASFITQYSTGQVSVEIEWELQKENSKRWNPEIQYTSNYNKSVNVDFTVDTNGVYSEPRPIGTRYLTRNL

SEQ ID NO: 60 - protein, 598 aa, synthetic construct
  source 1..598: note = Amino acid sequence of VP2 variant
TAPGKKRPVEHSPVEPDSSSGTGKAGQQPARKRLNFGQTGDADSVPDPQPLGQPPAAPSGLGTNTMATGSGAPMADNNEGADGVGNSSGNWHCDSTWMGDRVITTSTRTWALPTYNNHLYKQISSQSGASNDNHYFGYSTPWGYFDFNRFHCHFSPRDWQRLINNNWGFRPKRLNFKLFNIQVKEVTQNDGTTTIANNLTSTVQVFTDSEYQLPYVLGSAHQGCLPPFPADVFMVPQYGYLTLNNGSQAVGRSSFYCLEYFPSQMLRTGNNFTFSYTFEDVPFHSSYAHSQSLDRLMNPLIDQYLYYLSRTNTPSGTTTQSRLQFSQAGASDIRDQSRNWLPGPCYRQQRVSKTSADNNNSEYSWTGATKYHLNGRDSLVNPGPAMASHKDDEEKFFPQSGVLIFGKQGSEKTNVDIEKVMITDESEIAATNPVAYEQYGSVTTNLQNGNNQAATADVNTQGVLPGMVWQDRDVYLQGPIWAKIPHTDGHFHPSPLMGGFGLKHPPPQILIKNTPVPANPSTTFSAAKFASFITQYSTGQVSVEIEWELQKENSKRWNPEIQYTSNYNKSVNVDFTVDTNGVYSEPRPIGTRYLTRNL

SEQ ID NO: 61 - protein, 598 aa, synthetic construct
  source 1..598: note = Amino acid sequence of VP2 variant
TAPGKKRPVEHSPVEPDSSSGTGKAGQQPARKRLNFGQTGDADSVPDPQPLGQPPAAPSGLGTNTMATGSGAPMADNNEGADGVGNSSGNWHCDSTWMGDRVITTSTRTWALPTYNNHLYKQISSQSGASNDNHYFGYSTPWGYFDFNRFHCHFSPRDWQRLINNNWGFRPKRLNFKLFNIQVKEVTQNDGTTTIANNLTSTVQVFTDSEYQLPYVLGSAHQGCLPPFPADVFMVPQYGYLTLNNGSQAVGRSSFYCLEYFPSQMLRTGNNFTFSYTFEDVPFHSSYAHSQSLDRLMNPLIDQYLYYLSRTNTPSGTTTQSRLQFSQAGASDIRDQSRNWLPGPCYRQQRVSKTSADNNNSEYSWTGATKYHLNGRDSLVNPGPAMASHKDDEEKFFPQSGVLIFGKQGSEKTNVDIEKVMITDESEIAATNPVATEQYGCVATNLQRGYVQAATADVNTQGVLPGMVWQDRDVYLQGPIWAKIPHTDGHFHPSPLMGGFGLKHPPPQILIKNTPVPANPSTTFSAAKFASFITQYSTGQVSVEIEWELQKENSKRWNPEIQYTSNYNKSVNVDFTVDTNGVYSEPRPIGTRYLTRNL

SEQ ID NO: 62 - protein, 598 aa, synthetic construct
  source 1..598: note = Amino acid sequence of VP2 variant
TAPGKKRPVEHSPVEPDSSSGTGKAGQQPARKRLNFGQTGDADSVPDPQPLGQPPAAPSGLGTNTMATGSGAPMADNNEGADGVGNSSGNWHCDSTWMGDRVITTSTRTWALPTYNNHLYKQISSQSGASNDNHYFGYSTPWGYFDFNRFHCHFSPRDWQRLINNNWGFRPKRLNFKLFNIQVKEVTQNDGTTTIANNLTSTVQVFTDSEYQLPYVLGSAHQGCLPPFPADVFMVPQYGYLTLNNGSQAVGRSSFYCLEYFPSQMLRTGNNFTFSYTFEDVPFHSSYAHSQSLDRLMNPLIDQYLYYLSRTNTPSGTTTQSRLQFSQAGASDIRDQSRNWLPGPCYRQQRVSKTSADNNNSEYSWTGATKYHLNGRDSLVNPGPAMASHKDDEEKFFPQSGVLIFGKQGSEKTNVDIEKVMITDEQEVAATNPVATEQWGEVSTNLQRGNEQAATADVNTQGVLPGMVWQDRDVYLQGPIWAKIPHTDGHFHPSPLMGGFGLKHPPPQILIKNTPVPANPSTTFSAAKFASFITQYSTGQVSVEIEWELQKENSKRWNPEIQYTSNYNKSVNVDFTVDTNGVYSEPRPIGTRYLTRNL

SEQ ID NO: 63 - protein, 533 aa, synthetic construct
  source 1..533: note = Amino acid sequence of VP3 of wild-type AAV2
MATGSGAPMADNNEGADGVGNSSGNWHCDSTWMGDRVITTSTRTWALPTYNNHLYKQISSQSGASNDNHYFGYSTPWGYFDFNRFHCHFSPRDWQRLINNNWGFRPKRLNFKLFNIQVKEVTQNDGTTTIANNLTSTVQVFTDSEYQLPYVLGSAHQGCLPPFPADVFMVPQYGYLTLNNGSQAVGRSSFYCLEYFPSQMLRTGNNFTFSYTFEDVPFHSSYAHSQSLDRLMNPLIDQYLYYLSRTNTPSGTTTQSRLQFSQAGASDIRDQSRNWLPGPCYRQQRVSKTSADNNNSEYSWTGATKYHLNGRDSLVNPGPAMASHKDDEEKFFPQSGVLIFGKQGSEKTNVDIEKVMITDEEEIRTTNPVATEQYGSVSTNLQRGNRQAATADVNTQGVLPGMVWQDRDVYLQGPIWAKIPHTDGHFHPSPLMGGFGLKHPPPQILIKNTPVPANPSTTFSAAKFASFITQYSTGQVSVEIEWELQKENSKRWNPEIQYTSNYNKSVNVDFTVDTNGVYSEPRPIGTRYLTRNL

SEQ ID NO: 64 - protein, 533 aa, synthetic construct
  source 1..533: note = Amino acid sequence of VP3 variant
MATGSGAPMADNNEGADGVGNSSGNWHCDSTWMGDRVITTSTRTWALPTYNNHLYKQISSQSGASNDNHYFGYSTPWGYFDFNRFHCHFSPRDWQRLINNNWGFRPKRLNFKLFNIQVKEVTQNDGTTTIANNLTSTVQVFTDSEYQLPYVLGSAHQGCLPPFPADVFMVPQYGYLTLNNGSQAVGRSSFYCLEYFPSQMLRTGNNFTFSYTFEDVPFHSSYAHSQSLDRLMNPLIDQYLYYLSRTNTPSGTTTQSRLQFSQAGASDIRDQSRNWLPGPCYRQQRVSKTSADNNNSEYSWTGATKYHLNGRDSLVNPGPAMASHKDDEEKFFPQSGVLIFGKQGSEKTNVDIEKVMITDEEEIAATNPVATESYGEVATNLQRGNVQAATADVNTQGVLPGMVWQDRDVYLQGPIWAKIPHTDGHFHPSPLMGGFGLKHPPPQILIKNTPVPANPSTTFSAAKFASFITQYSTGQVSVEIEWELQKENSKRWNPEIQYTSNYNKSVNVDFTVDTNGVYSEPRPIGTRYLTRNL

SEQ ID NO: 65 - protein, 533 aa, synthetic construct
  source 1..533: note = Amino acid sequence of VP3 variant
MATGSGAPMADNNEGADGVGNSSGNWHCDSTWMGDRVITTSTRTWALPTYNNHLYKQISSQSGASNDNHYFGYSTPWGYFDFNRFHCHFSPRDWQRLINNNWGFRPKRLNFKLFNIQVKEVTQNDGTTTIANNLTSTVQVFTDSEYQLPYVLGSAHQGCLPPFPADVFMVPQYGYLTLNNGSQAVGRSSFYCLEYFPSQMLRTGNNFTFSYTFEDVPFHSSYAHSQSLDRLMNPLIDQYLYYLSRTNTPSGTTTQSRLQFSQAGASDIRDQSRNWLPGPCYRQQRVSKTSADNNNSEYSWTGATKYHLNGRDSLVNPGPAMASHKDDEEKFFPQSGVLIFGKQGSEKTNVDIEKVMITDEQEVAATNPVATESWGSVSTNLQRGNTQAATADVNTQGVLPGMVWQDRDVYLQGPIWAKIPHTDGHFHPSPLMGGFGLKHPPPQILIKNTPVPANPSTTFSAAKFASFITQYSTGQVSVEIEWELQKENSKRWNPEIQYTSNYNKSVNVDFTVDTNGVYSEPRPIGTRYLTRNL

SEQ ID NO: 66 - protein, 533 aa, synthetic construct
  source 1..533: note = Amino acid sequence of VP3 variant
MATGSGAPMADNNEGADGVGNSSGNWHCDSTWMGDRVITTSTRTWALPTYNNHLYKQISSQSGASNDNHYFGYSTPWGYFDFNRFHCHFSPRDWQRLINNNWGFRPKRLNFKLFNIQVKEVTQNDGTTTIANNLTSTVQVFTDSEYQLPYVLGSAHQGCLPPFPADVFMVPQYGYLTLNNGSQAVGRSSFYCLEYFPSQMLRTGNNFTFSYTFEDVPFHSSYAHSQSLDRLMNPLIDQYLYYLSRTNTPSGTTTQSRLQFSQAGASDIRDQSRNWLPGPCYRQQRVSKTSADNNNSEYSWTGATKYHLNGRDSLVNPGPAMASHKDDEEKFFPQSGVLIFGKQGSEKTNVDIEKVMITDESEIRTTNPIATEQWGSVSTNLQNGNRQAATADVNTQGVLPGMVWQDRDVYLQGPIWAKIPHTDGHFHPSPLMGGFGLKHPPPQILIKNTPVPANPSTTFSAAKFASFITQYSTGQVSVEIEWELQKENSKRWNPEIQYTSNYNKSVNVDFTVDTNGVYSEPRPIGTRYLTRNL

SEQ ID NO: 67 - protein, 533 aa, synthetic construct
  source 1..533: note = Amino acid sequence of VP3 variant
MATGSGAPMADNNEGADGVGNSSGNWHCDSTWMGDRVITTSTRTWALPTYNNHLYKQISSQSGASNDNHYFGYSTPWGYFDFNRFHCHFSPRDWQRLINNNWGFRPKRLNFKLFNIQVKEVTQNDGTTTIANNLTSTVQVFTDSEYQLPYVLGSAHQGCLPPFPADVFMVPQYGYLTLNNGSQAVGRSSFYCLEYFPSQMLRTGNNFTFSYTFEDVPFHSSYAHSQSLDRLMNPLIDQYLYYLSRTNTPSGTTTQSRLQFSQAGASDIRDQSRNWLPGPCYRQQRVSKTSADNNNSEYSWTGATKYHLNGRDSLVNPGPAMASHKDDEEKFFPQSGVLIFGKQGSEKTNVDIEKVMITDEEEIATTNPVATEQWGSVSTNLQRGATQAATADVNTQGVLPGMVWQDRDVYLQGPIWAKIPHTDGHFHPSPLMGGFGLKHPPPQILIKNTPVPANPSTTFSAAKFASFITQYSTGQVSVEIEWELQKENSKRWNPEIQYTSNYNKSVNVDFTVDTNGVYSEPRPIGTRYLTRNL

SEQ ID NO: 68 - protein, 533 aa, synthetic construct
  source 1..533: note = Amino acid sequence of VP3 variant
MATGSGAPMADNNEGADGVGNSSGNWHCDSTWMGDRVITTSTRTWALPTYNNHLYKQISSQSGASNDNHYFGYSTPWGYFDFNRFHCHFSPRDWQRLINNNWGFRPKRLNFKLFNIQVKEVTQNDGTTTIANNLTSTVQVFTDSEYQLPYVLGSAHQGCLPPFPADVFMVPQYGYLTLNNGSQAVGRSSFYCLEYFPSQMLRTGNNFTFSYTFEDVPFHSSYAHSQSLDRLMNPLIDQYLYYLSRTNTPSGTTTQSRLQFSQAGASDIRDQSRNWLPGPCYRQQRVSKTSADNNNSEYSWTGATKYHLNGRDSLVNPGPAMASHKDDEEKFFPQSGVLIFGKQGSEKTNVDIEKVMITDESEIATTNPVATESYGEVSTNLQRNPVQAATADVNTQGVLPGMVWQDRDVYLQGPIWAKIPHTDGHFHPSPLMGGFGLKHPPPQILIKNTPVPANPSTTFSAAKFASFITQYSTGQVSVEIEWELQKENSKRWNPEIQYTSNYNKSVNVDFTVDTNGVYSEPRPIGTRYLTRNL

SEQ ID NO: 69 - protein, 533 aa, synthetic construct
  source 1..533: note = Amino acid sequence of VP3 variant
MATGSGAPMADNNEGADGVGNSSGNWHCDSTWMGDRVITTSTRTWALPTYNNHLYKQISSQSGASNDNHYFGYSTPWGYFDFNRFHCHFSPRDWQRLINNNWGFRPKRLNFKLFNIQVKEVTQNDGTTTIANNLTSTVQVFTDSEYQLPYVLGSAHQGCLPPFPADVFMVPQYGYLTLNNGSQAVGRSSFYCLEYFPSQMLRTGNNFTFSYTFEDVPFHSSYAHSQSLDRLMNPLIDQYLYYLSRTNTPSGTTTQSRLQFSQAGASDIRDQSRNWLPGPCYRQQRVSKTSADNNNSEYSWTGATKYHLNGRDSLVNPGPAMASHKDDEEKFFPQSGVLIFGKQGSEKTNVDIEKVMITDEEEIRTTNPVAYEQYGVVATNLQNSNAQAATADVNTQGVLPGMVWQDRDVYLQGPIWAKIPHTDGHFHPSPLMGGFGLKHPPPQILIKNTPVPANPSTTFSAAKFASFITQYSTGQVSVEIEWELQKENSKRWNPEIQYTSNYNKSVNVDFTVDTNGVYSEPRPIGTRYLTRNL

SEQ ID NO: 70 - protein, 533 aa, synthetic construct
  source 1..533: note = Amino acid sequence of VP3 variant
MATGSGAPMADNNEGADGVGNSSGNWHCDSTWMGDRVITTSTRTWALPTYNNHLYKQISSQSGASNDNHYFGYSTPWGYFDFNRFHCHFSPRDWQRLINNNWGFRPKRLNFKLFNIQVKEVTQNDGTTTIANNLTSTVQVFTDSEYQLPYVLGSAHQGCLPPFPADVFMVPQYGYLTLNNGSQAVGRSSFYCLEYFPSQMLRTGNNFTFSYTFEDVPFHSSYAHSQSLDRLMNPLIDQYLYYLSRTNTPSGTTTQSRLQFSQAGASDIRDQSRNWLPGPCYRQQRVSKTSADNNNSEYSWTGATKYHLNGRDSLVNPGPAMASHKDDEEKFFPQSGVLIFGKQGSEKTNVDIEKVMITDEAEIATTNPVAAEQYGEVSTNLQNGNRQAATADVNTQGVLPGMVWQDRDVYLQGPIWAKIPHTDGHFHPSPLMGGFGLKHPPPQILIKNTPVPANPSTTFSAAKFASFITQYSTGQVSVEIEWELQKENSKRWNPEIQYTSNYNKSVNVDFTVDTNGVYSEPRPIGTRYLTRNL

SEQ ID NO: 71 - protein, 533 aa, synthetic construct
  source 1..533: note = Amino acid sequence of VP3 variant
MATGSGAPMADNNEGADGVGNSSGNWHCDSTWMGDRVITTSTRTWALPTYNNHLYKQISSQSGASNDNHYFGYSTPWGYFDFNRFHCHFSPRDWQRLINNNWGFRPKRLNFKLFNIQVKEVTQNDGTTTIANNLTSTVQVFTDSEYQLPYVLGSAHQGCLPPFPADVFMVPQYGYLTLNNGSQAVGRSSFYCLEYFPSQMLRTGNNFTFSYTFEDVPFHSSYAHSQSLDRLMNPLIDQYLYYLSRTNTPSGTTTQSRLQFSQAGASDIRDQSRNWLPGPCYRQQRVSKTSADNNNSEYSWTGATKYHLNGRDSLVNPGPAMASHKDDEEKFFPQSGVLIFGKQGSEKTNVDIEKVMITDEQEVAATNPVATEHYGQVATNLQTGNRQAATADVNTQGVLPGMVWQDRDVYLQGPIWAKIPHTDGHFHPSPLMGGFGLKHPPPQILIKNTPVPANPSTTFSAAKFASFITQYSTGQVSVEIEWELQKENSKRWNPEIQYTSNYNKSVNVDFTVDTNGVYSEPRPIGTRYLTRNL

SEQ ID NO: 72 - protein, 533 aa, synthetic construct
  source 1..533: note = Amino acid sequence of VP3 variant
MATGSGAPMADNNEGADGVGNSSGNWHCDSTWMGDRVITTSTRTWALPTYNNHLYKQISSQSGASNDNHYFGYSTPWGYFDFNRFHCHFSPRDWQRLINNNWGFRPKRLNFKLFNIQVKEVTQNDGTTTIANNLTSTVQVFTDSEYQLPYVLGSAHQGCLPPFPADVFMVPQYGYLTLNNGSQAVGRSSFYCLEYFPSQMLRTGNNFTFSYTFEDVPFHSSYAHSQSLDRLMNPLIDQYLYYLSRTNTPSGTTTQSRLQFSQAGASDIRDQSRNWLPGPCYRQQRVSKTSADNNNSEYSWTGATKYHLNGRDSLVNPGPAMASHKDDEEKFFPQSGVLIFGKQGSEKTNVDIEKVMITDEEEINTTNPVYTEQYGSVSTNLQRGNIQAATADVNTQGVLPGMVWQDRDVYLQGPIWAKIPHTDGHFHPSPLMGGFGLKHPPPQILIKNTPVPANPSTTFSAAKFASFITQYSTGQVSVEIEWELQKENSKRWNPEIQYTSNYNKSVNVDFTVDTNGVYSEPRPIGTRYLTRNL

SEQ ID NO: 73 - protein, 533 aa, synthetic construct
  source 1..533: note = Amino acid sequence of VP3 variant
MATGSGAPMADNNEGADGVGNSSGNWHCDSTWMGDRVITTSTRTWALPTYNNHLYKQISSQSGASNDNHYFGYSTPWGYFDFNRFHCHFSPRDWQRLINNNWGFRPKRLNFKLFNIQVKEVTQNDGTTTIANNLTSTVQVFTDSEYQLPYVLGSAHQGCLPPFPADVFMVPQYGYLTLNNGSQAVGRSSFYCLEYFPSQMLRTGNNFTFSYTFEDVPFHSSYAHSQSLDRLMNPLIDQYLYYLSRTNTPSGTTTQSRLQFSQAGASDIRDQSRNWLPGPCYRQQRVSKTSADNNNSEYSWTGATKYHLNGRDSLVNPGPAMASHKDDEEKFFPQSGVLIFGKQGSEKTNVDIEKVMITDEQEVAATNPVADEQYGVVATNLQRGNVQAATADVNTQGVLPGMVWQDRDVYLQGPIWAKIPHTDGHFHPSPLMGGFGLKHPPPQILIKNTPVPANPSTTFSAAKFASFITQYSTGQVSVEIEWELQKENSKRWNPEIQYTSNYNKSVNVDFTVDTNGVYSEPRPIGTRYLTRNL

SEQ ID NO: 74 - protein, 533 aa, synthetic construct
  source 1..533: note = Amino acid sequence of VP3 variant
MATGSGAPMADNNEGADGVGNSSGNWHCDSTWMGDRVITTSTRTWALPTYNNHLYKQISSQSGASNDNHYFGYSTPWGYFDFNRFHCHFSPRDWQRLINNNWGFRPKRLNFKLFNIQVKEVTQNDGTTTIANNLTSTVQVFTDSEYQLPYVLGSAHQGCLPPFPADVFMVPQYGYLTLNNGSQAVGRSSFYCLEYFPSQMLRTGNNFTFSYTFEDVPFHSSYAHSQSLDRLMNPLIDQYLYYLSRTNTPSGTTTQSRLQFSQAGASDIRDQSRNWLPGPCYRQQRVSKTSADNNNSEYSWTGATKYHLNGRDSLVNPGPAMASHKDDEEKFFPQSGVLIFGKQGSEKTNVDIEKVMITDESEIAATNPVATEQWGSVATNRQRGETQAATADVNTQGVLPGMVWQDRDVYLQGPIWAKIPHTDGHFHPSPLMGGFGLKHPPPQILIKNTPVPANPSTTFSAAKFASFITQYSTGQVSVEIEWELQKENSKRWNPEIQYTSNYNKSVNVDFTVDTNGVYSEPRPIGTRYLTRNL

SEQ ID NO: 75 - protein, 533 aa, synthetic construct
  source 1..533: note = Amino acid sequence of VP3 variant
MATGSGAPMADNNEGADGVGNSSGNWHCDSTWMGDRVITTSTRTWALPTYNNHLYKQISSQSGASNDNHYFGYSTPWGYFDFNRFHCHFSPRDWQRLINNNWGFRPKRLNFKLFNIQVKEVTQNDGTTTIANNLTSTVQVFTDSEYQLPYVLGSAHQGCLPPFPADVFMVPQYGYLTLNNGSQAVGRSSFYCLEYFPSQMLRTGNNFTFSYTFEDVPFHSSYAHSQSLDRLMNPLIDQYLYYLSRTNTPSGTTTQSRLQFSQAGASDIRDQSRNWLPGPCYRQQRVSKTSADNNNSEYSWTGATKYHLNGRDSLVNPGPAMASHKDDEEKFFPQSGVLIFGKQGSEKTNVDIEKVMITDEQEVAATNPVATEQWGEVSTNLQRSTTQAATADVNTQGVLPGMVWQDRDVYLQGPIWAKIPHTDGHFHPSPLMGGFGLKHPPPQILIKNTPVPANPSTTFSAAKFASFITQYSTGQVSVEIEWELQKENSKRWNPEIQYTSNYNKSVNVDFTVDTNGVYSEPRPIGTRYLTRNL

SEQ ID NO: 76 - protein, 533 aa, synthetic construct
  source 1..533: note = Amino acid sequence of VP3 variant
MATGSGAPMADNNEGADGVGNSSGNWHCDSTWMGDRVITTSTRTWALPTYNNHLYKQISSQSGASNDNHYFGYSTPWGYFDFNRFHCHFSPRDWQRLINNNWGFRPKRLNFKLFNIQVKEVTQNDGTTTIANNLTSTVQVFTDSEYQLPYVLGSAHQGCLPPFPADVFMVPQYGYLTLNNGSQAVGRSSFYCLEYFPSQMLRTGNNFTFSYTFEDVPFHSSYAHSQSLDRLMNPLIDQYLYYLSRTNTPSGTTTQSRLQFSQAGASDIRDQSRNWLPGPCYRQQRVSKTSADNNNSEYSWTGATKYHLNGRDSLVNPGPAMASHKDDEEKFFPQSGVLIFGKQGSEKTNVDIEKVMITQESEIAATNPVATEQWGVVATNLQNGTRQAATADVNTQGVLPGMVWQDRDVYLQGPIWAKIPHTDGHFHPSPLMGGFGLKHPPPQILIKNTPVPANPSTTFSAAKFASFITQYSTGQVSVEIEWELQKENSKRWNPEIQYTSNYNKSVNVDFTVDTNGVYSEPRPIGTRYLTRNL

SEQ ID NO: 77 - protein, 533 aa, synthetic construct
  source 1..533: note = Amino acid sequence of VP3 variant
MATGSGAPMADNNEGADGVGNSSGNWHCDSTWMGDRVITTSTRTWALPTYNNHLYKQISSQSGASNDNHYFGYSTPWGYFDFNRFHCHFSPRDWQRLINNNWGFRPKRLNFKLFNIQVKEVTQNDGTTTIANNLTSTVQVFTDSEYQLPYVLGSAHQGCLPPFPADVFMVPQYGYLTLNNGSQAVGRSSFYCLEYFPSQMLRTGNNFTFSYTFEDVPFHSSYAHSQSLDRLMNPLIDQYLYYLSRTNTPSGTTTQSRLQFSQAGASDIRDQSRNWLPGPCYRQQRVSKTSADNNNSEYSWTGATKYHLNGRDSLVNPGPAMASHKDDEEKFFPQSGVLIFGKQGSEKTNVDIEKVMITDESEVAATNPVATEQWGEVSTNNQRGTTQAATADVNTQGVLPGMVWQDRDVYLQGPIWAKIPHTDGHFHPSPLMGGFGLKHPPPQILIKNTPVPANPSTTFSAAKFASFITQYSTGQVSVEIEWELQKENSKRWNPEIQYTSNYNKSVNVDFTVDTNGVYSEPRPIGTRYLTRNL

SEQ ID NO: 78 - protein, 533 aa, synthetic construct
  source 1..533: note = Amino acid sequence of VP3 variant
MATGSGAPMADNNEGADGVGNSSGNWHCDSTWMGDRVITTSTRTWALPTYNNHLYKQISSQSGASNDNHYFGYSTPWGYFDFNRFHCHFSPRDWQRLINNNWGFRPKRLNFKLFNIQVKEVTQNDGTTTIANNLTSTVQVFTDSEYQLPYVLGSAHQGCLPPFPADVFMVPQYGYLTLNNGSQAVGRSSFYCLEYFPSQMLRTGNNFTFSYTFEDVPFHSSYAHSQSLDRLMNPLIDQYLYYLSRTNTPSGTTTQSRLQFSQAGASDIRDQSRNWLPGPCYRQQRVSKTSADNNNSEYSWTGATKYHLNGRDSLVNPGPAMASHKDDEEKFFPQSGVLIFGKQGSEKTNVDIEKVMITDEEEIRTTNPVATEQYGSVSTNIQHGNRQAATADVNTQGVLPGMVWQDRDVYLQGPIWAKIPHTDGHFHPSPLMGGFGLKHPPPQILIKNTPVPANPSTTFSAAKFASFITQYSTGQVSVEIEWELQKENSKRWNPEIQYTSNYNKSVNVDFTVDTNGVYSEPRPIGTRYLTRNL

SEQ ID NO: 79 - protein, 533 aa, synthetic construct
  source 1..533: note = Amino acid sequence of VP3 variant
MATGSGAPMADNNEGADGVGNSSGNWHCDSTWMGDRVITTSTRTWALPTYNNHLYKQISSQSGASNDNHYFGYSTPWGYFDFNRFHCHFSPRDWQRLINNNWGFRPKRLNFKLFNIQVKEVTQNDGTTTIANNLTSTVQVFTDSEYQLPYVLGSAHQGCLPPFPADVFMVPQYGYLTLNNGSQAVGRSSFYCLEYFPSQMLRTGNNFTFSYTFEDVPFHSSYAHSQSLDRLMNPLIDQYLYYLSRTNTPSGTTTQSRLQFSQAGASDIRDQSRNWLPGPCYRQQRVSKTSADNNNSEYSWTGATKYHLNGRDSLVNPGPAMASHKDDEEKFFPQSGVLIFGKQGSEKTNVDIEKVMITDEEEIRTTNPVATEQYGSVSTWLQRGNRQAATADVNTQGVLPGMVWQDRDVYLQGPIWAKIPHTDGHFHPSPLMGGFGLKHPPPQILIKNTPVPANPSTTFSAAKFASFITQYSTGQVSVEIEWELQKENSKRWNPEIQYTSNYNKSVNVDFTVDTNGVYSEPRPIGTRYLTRNL

SEQ ID NO: 80 - protein, 533 aa, synthetic construct
  source 1..533: note = Amino acid sequence of VP3 variant
MATGSGAPMADNNEGADGVGNSSGNWHCDSTWMGDRVITTSTRTWALPTYNNHLYKQISSQSGASNDNHYFGYSTPWGYFDFNRFHCHFSPRDWQRLINNNWGFRPKRLNFKLFNIQVKEVTQNDGTTTIANNLTSTVQVFTDSEYQLPYVLGSAHQGCLPPFPADVFMVPQYGYLTLNNGSQAVGRSSFYCLEYFPSQMLRTGNNFTFSYTFEDVPFHSSYAHSQSLDRLMNPLIDQYLYYLSRTNTPSGTTTQSRLQFSQAGASDIRDQSRNWLPGPCYRQQRVSKTSADNNNSEYSWTGATKYHLNGRDSLVNPGPAMASHKDDEEKFFPQSGVLIFGKQGSEKTNVDIEKVMITDEQEIAATNPVATEQYGEVSTNLQNQNRQAATADVNTQGVLPGMVWQDRDVYLQGPIWAKIPHTDGHFHPSPLMGGFGLKHPPPQILIKNTPVPANPSTTFSAAKFASFITQYSTGQVSVEIEWELQKENSKRWNPEIQYTSNYNKSVNVDFTVDTNGVYSEPRPIGTRYLTRNL

SEQ ID NO: 81 - protein, 533 aa, synthetic construct
  source 1..533: note = Amino acid sequence of VP3 variant
MATGSGAPMADNNEGADGVGNSSGNWHCDSTWMGDRVITTSTRTWALPTYNNHLYKQISSQSGASNDNHYFGYSTPWGYFDFNRFHCHFSPRDWQRLINNNWGFRPKRLNFKLFNIQVKEVTQNDGTTTIANNLTSTVQVFTDSEYQLPYVLGSAHQGCLPPFPADVFMVPQYGYLTLNNGSQAVGRSSFYCLEYFPSQMLRTGNNFTFSYTFEDVPFHSSYAHSQSLDRLMNPLIDQYLYYLSRTNTPSGTTTQSRLQFSQAGASDIRDQSRNWLPGPCYRQQRVSKTSADNNNSEYSWTGATKYHLNGRDSLVNPGPAMASHKDDEEKFFPQSGVLIFGKQGSEKTNVDIEKVMITQESEIAATNPVATEQWGEVATNLQRGTTQAATADVNTQGVLPGMVWQDRDVYLQGPIWAKIPHTDGHFHPSPLMGGFGLKHPPPQILIKNTPVPANPSTTFSAAKFASFITQYSTGQVSVEIEWELQKENSKRWNPEIQYTSNYNKSVNVDFTVDTNGVYSEPRPIGTRYLTRNL

SEQ ID NO: 82 - protein, 533 aa, synthetic construct
  source 1..533: note = Amino acid sequence of VP3 variant
MATGSGAPMADNNEGADGVGNSSGNWHCDSTWMGDRVITTSTRTWALPTYNNHLYKQISSQSGASNDNHYFGYSTPWGYFDFNRFHCHFSPRDWQRLINNNWGFRPKRLNFKLFNIQVKEVTQNDGTTTIANNLTSTVQVFTDSEYQLPYVLGSAHQGCLPPFPADVFMVPQYGYLTLNNGSQAVGRSSFYCLEYFPSQMLRTGNNFTFSYTFEDVPFHSSYAHSQSLDRLMNPLIDQYLYYLSRTNTPSGTTTQSRLQFSQAGASDIRDQSRNWLPGPCYRQQRVSKTSADNNNSEYSWTGATKYHLNGRDSLVNPGPAMASHKDDEEKFFPQSGVLIFGKQGSEKTNVDIEKVMITDEWEIRTTNPVATEQYGSVSTNLQRLNRQAATADVNTQGVLPGMVWQDRDVYLQGPIWAKIPHTDGHFHPSPLMGGFGLKHPPPQILIKNTPVPANPSTTFSAAKFASFITQYSTGQVSVEIEWELQKENSKRWNPEIQYTSNYNKSVNVDFTVDTNGVYSEPRPIGTRYLTRNL

SEQ ID NO: 83 - protein, 533 aa, synthetic construct
  source 1..533: note = Amino acid sequence of VP3 variant
MATGSGAPMADNNEGADGVGNSSGNWHCDSTWMGDRVITTSTRTWALPTYNNHLYKQISSQSGASNDNHYFGYSTPWGYFDFNRFHCHFSPRDWQRLINNNWGFRPKRLNFKLFNIQVKEVTQNDGTTTIANNLTSTVQVFTDSEYQLPYVLGSAHQGCLPPFPADVFMVPQYGYLTLNNGSQAVGRSSFYCLEYFPSQMLRTGNNFTFSYTFEDVPFHSSYAHSQSLDRLMNPLIDQYLYYLSRTNTPSGTTTQSRLQFSQAGASDIRDQSRNWLPGPCYRQQRVSKTSADNNNSEYSWTGATKYHLNGRDSLVNPGPAMASHKDDEEKFFPQSGVLIFGKQGSEKTNVDIEKVMITDEAEIAATNPVATEQWGEVSTNTQNGARQAATADVNTQGVLPGMVWQDRDVYLQGPIWAKIPHTDGHFHPSPLMGGFGLKHPPPQILIKNTPVPANPSTTFSAAKFASFITQYSTGQVSVEIEWELQKENSKRWNPEIQYTSNYNKSVNVDFTVDTNGVYSEPRPIGTRYLTRNL

SEQ ID NO: 84 - protein, 533 aa, synthetic construct
  source 1..533: note = Amino acid sequence of VP3 variant
MATGSGAPMADNNEGADGVGNSSGNWHCDSTWMGDRVITTSTRTWALPTYNNHLYKQISSQSGASNDNHYFGYSTPWGYFDFNRFHCHFSPRDWQRLINNNWGFRPKRLNFKLFNIQVKEVTQNDGTTTIANNLTSTVQVFTDSEYQLPYVLGSAHQGCLPPFPADVFMVPQYGYLTLNNGSQAVGRSSFYCLEYFPSQMLRTGNNFTFSYTFEDVPFHSSYAHSQSLDRLMNPLIDQYLYYLSRTNTPSGTTTQSRLQFSQAGASDIRDQSRNWLPGPCYRQQRVSKTSADNNNSEYSWTGATKYHLNGRDSLVNPGPAMASHKDDEEKFFPQSGVLIFGKQGSEKTNVDIEKVMITDEQEVAATNPVATEAYGTVSTNLQRQNTQAATADVNTQGVLPGMVWQDRDVYLQGPIWAKIPHTDGHFHPSPLMGGFGLKHPPPQILIKNTPVPANPSTTFSAAKFASFITQYSTGQVSVEIEWELQKENSKRWNPEIQYTSNYNKSVNVDFTVDTNGVYSEPRPIGTRYLTRNL

SEQ ID NO: 85 - protein, 533 aa, synthetic construct
  source 1..533: note = Amino acid sequence of VP3 variant
MATGSGAPMADNNEGADGVGNSSGNWHCDSTWMGDRVITTSTRTWALPTYNNHLYKQISSQSGASNDNHYFGYSTPWGYFDFNRFHCHFSPRDWQRLINNNWGFRPKRLNFKLFNIQVKEVTQNDGTTTIANNLTSTVQVFTDSEYQLPYVLGSAHQGCLPPFPADVFMVPQYGYLTLNNGSQAVGRSSFYCLEYFPSQMLRTGNNFTFSYTFEDVPFHSSYAHSQSLDRLMNPLIDQYLYYLSRTNTPSGTTTQSRLQFSQAGASDIRDQSRNWLPGPCYRQQRVSKTSADNNNSEYSWTGATKYHLNGRDSLVNPGPAMASHKDDEEKFFPQSGVLIFGKQGSEKTNVDIEKVMITDEAEIAATNPVATEQYGTVSTNLQTGNQQAATADVNTQGVLPGMVWQDRDVYLQGPIWAKIPHTDGHFHPSPLMGGFGLKHPPPQILIKNTPVPANPSTTFSAAKFASFITQYSTGQVSVEIEWELQKENSKRWNPEIQYTSNYNKSVNVDFTVDTNGVYSEPRPIGTRYLTRNL

SEQ ID NO: 86 - protein, 533 aa, synthetic construct
  source 1..533: note = Amino acid sequence of VP3 variant
MATGSGAPMADNNEGADGVGNSSGNWHCDSTWMGDRVITTSTRTWALPTYNNHLYKQISSQSGASNDNHYFGYSTPWGYFDFNRFHCHFSPRDWQRLINNNWGFRPKRLNFKLFNIQVKEVTQNDGTTTIANNLTSTVQVFTDSEYQLPYVLGSAHQGCLPPFPADVFMVPQYGYLTLNNGSQAVGRSSFYCLEYFPSQMLRTGNNFTFSYTFEDVPFHSSYAHSQSLDRLMNPLIDQYLYYLSRTNTPSGTTTQSRLQFSQAGASDIRDQSRNWLPGPCYRQQRVSKTSADNNNSEYSWTGATKYHLNGRDSLVNPGPAMASHKDDEEKFFPQSGVLIFGKQGSEKTNVDIEKVMITDESEIRTTNPVATESYGEVATNLQTGTTQAATADVNTQGVLPGMVWQDRDVYLQGPIWAKIPHTDGHFHPSPLMGGFGLKHPPPQILIKNTPVPANPSTTFSAAKFASFITQYSTGQVSVEIEWELQKENSKRWNPEIQYTSNYNKSVNVDFTVDTNGVYSEPRPIGTRYLTRNL

SEQ ID NO: 87 - protein, 533 aa, synthetic construct
  source 1..533: note = Amino acid sequence of VP3 variant
MATGSGAPMADNNEGADGVGNSSGNWHCDSTWMGDRVITTSTRTWALPTYNNHLYKQISSQSGASNDNHYFGYSTPWGYFDFNRFHCHFSPRDWQRLINNNWGFRPKRLNFKLFNIQVKEVTQNDGTTTIANNLTSTVQVFTDSEYQLPYVLGSAHQGCLPPFPADVFMVPQYGYLTLNNGSQAVGRSSFYCLEYFPSQMLRTGNNFTFSYTFEDVPFHSSYAHSQSLDRLMNPLIDQYLYYLSRTNTPSGTTTQSRLQFSQAGASDIRDQSRNWLPGPCYRQQRVSKTSADNNNSEYSWTGATKYHLNGRDSLVNPGPAMASHKDDEEKFFPQSGVLIFGKQGSEKTNVDIEKVMITDEAEIATTNPVATEQWGSVSTNLQGGNLQAATADVNTQGVLPGMVWQDRDVYLQGPIWAKIPHTDGHFHPSPLMGGFGLKHPPPQILIKNTPVPANPSTTFSAAKFASFITQYSTGQVSVEIEWELQKENSKRWNPEIQYTSNYNKSVNVDFTVDTNGVYSEPRPIGTRYLTRNL

SEQ ID NO: 88 - protein, 533 aa, synthetic construct
  source 1..533: note = Amino acid sequence of VP3 variant
MATGSGAPMADNNEGADGVGNSSGNWHCDSTWMGDRVITTSTRTWALPTYNNHLYKQISSQSGASNDNHYFGYSTPWGYFDFNRFHCHFSPRDWQRLINNNWGFRPKRLNFKLFNIQVKEVTQNDGTTTIANNLTSTVQVFTDSEYQLPYVLGSAHQGCLPPFPADVFMVPQYGYLTLNNGSQAVGRSSFYCLEYFPSQMLRTGNNFTFSYTFEDVPFHSSYAHSQSLDRLMNPLIDQYLYYLSRTNTPSGTTTQSRLQFSQAGASDIRDQSRNWLPGPCYRQQRVSKTSADNNNSEYSWTGATKYHLNGRDSLVNPGPAMASHKDDEEKFFPQSGVLIFGKQGSEKTNVDIEKVMITNESEIAATNPVATEQYGVVATNLQNGTVQAATADVNTQGVLPGMVWQDRDVYLQGPIWAKIPHTDGHFHPSPLMGGFGLKHPPPQILIKNTPVPANPSTTFSAAKFASFITQYSTGQVSVEIEWELQKENSKRWNPEIQYTSNYNKSVNVDFTVDTNGVYSEPRPIGTRYLTRNL

SEQ ID NO: 89 - protein, 533 aa, synthetic construct
  source 1..533: note = Amino acid sequence of VP3 variant
MATGSGAPMADNNEGADGVGNSSGNWHCDSTWMGDRVITTSTRTWALPTYNNHLYKQISSQSGASNDNHYFGYSTPWGYFDFNRFHCHFSPRDWQRLINNNWGFRPKRLNFKLFNIQVKEVTQNDGTTTIANNLTSTVQVFTDSEYQLPYVLGSAHQGCLPPFPADVFMVPQYGYLTLNNGSQAVGRSSFYCLEYFPSQMLRTGNNFTFSYTFEDVPFHSSYAHSQSLDRLMNPLIDQYLYYLSRTNTPSGTTTQSRLQFSQAGASDIRDQSRNWLPGPCYRQQRVSKTSADNNNSEYSWTGATKYHLNGRDSLVNPGPAMASHKDDEEKFFPQSGVLIFGKQGSEKTNVDIEKVMITDESEIRTTNPVATEQWGEVATNLQNGNIQAATADVNTQGVLPGMVWQDRDVYLQGPIWAKIPHTDGHFHPSPLMGGFGLKHPPPQILIKNTPVPANPSTTFSAAKFASFITQYSTGQVSVEIEWELQKENSKRWNPEIQYTSNYNKSVNVDFTVDTNGVYSEPRPIGTRYLTRNL

SEQ ID NO: 90 - protein, 533 aa, synthetic construct
  source 1..533: note = Amino acid sequence of VP3 variant
MATGSGAPMADNNEGADGVGNSSGNWHCDSTWMGDRVITTSTRTWALPTYNNHLYKQISSQSGASNDNHYFGYSTPWGYFDFNRFHCHFSPRDWQRLINNNWGFRPKRLNFKLFNIQVKEVTQNDGTTTIANNLTSTVQVFTDSEYQLPYVLGSAHQGCLPPFPADVFMVPQYGYLTLNNGSQAVGRSSFYCLEYFPSQMLRTGNNFTFSYTFEDVPFHSSYAHSQSLDRLMNPLIDQYLYYLSRTNTPSGTTTQSRLQFSQAGASDIRDQSRNWLPGPCYRQQRVSKTSADNNNSEYSWTGATKYHLNGRDSLVNPGPAMASHKDDEEKFFPQSGVLIFGKQGSEKTNVDIEKVMITDEAEIAATNPVATEQYGCVASNIQNSNTQAATADVNTQGVLPGMVWQDRDVYLQGPIWAKIPHTDGHFHPSPLMGGFGLKHPPPQILIKNTPVPANPSTTFSAAKFASFITQYSTGQVSVEIEWELQKENSKRWNPEIQYTSNYNKSVNVDFTVDTNGVYSEPRPIGTRYLTRNL

SEQ ID NO: 91 - protein, 533 aa, synthetic construct
  source 1..533: note = Amino acid sequence of VP3 variant
MATGSGAPMADNNEGADGVGNSSGNWHCDSTWMGDRVITTSTRTWALPTYNNHLYKQISSQSGASNDNHYFGYSTPWGYFDFNRFHCHFSPRDWQRLINNNWGFRPKRLNFKLFNIQVKEVTQNDGTTTIANNLTSTVQVFTDSEYQLPYVLGSAHQGCLPPFPADVFMVPQYGYLTLNNGSQAVGRSSFYCLEYFPSQMLRTGNNFTFSYTFEDVPFHSSYAHSQSLDRLMNPLIDQYLYYLSRTNTPSGTTTQSRLQFSQAGASDIRDQSRNWLPGPCYRQQRVSKTSADNNNSEYSWTGATKYHLNGRDSLVNPGPAMASHKDDEEKFFPQSGVLIFGKQGSEKTNVDIEKVMITDESEIAATNPVAYEQYGSVTTNLQNGNNQAATADVNTQGVLPGMVWQDRDVYLQGPIWAKIPHTDGHFHPSPLMGGFGLKHPPPQILIKNTPVPANPSTTFSAAKFASFITQYSTGQVSVEIEWELQKENSKRWNPEIQYTSNYNKSVNVDFTVDTNGVYSEPRPIGTRYLTRNL

SEQ ID NO: 92 - protein, 533 aa, synthetic construct
  source 1..533: note = Amino acid sequence of VP3 variant
MATGSGAPMADNNEGADGVGNSSGNWHCDSTWMGDRVITTSTRTWALPTYNNHLYKQISSQSGASNDNHYFGYSTPWGYFDFNRFHCHFSPRDWQRLINNNWGFRPKRLNFKLFNIQVKEVTQNDGTTTIANNLTSTVQVFTDSEYQLPYVLGSAHQGCLPPFPADVFMVPQYGYLTLNNGSQAVGRSSFYCLEYFPSQMLRTGNNFTFSYTFEDVPFHSSYAHSQSLDRLMNPLIDQYLYYLSRTNTPSGTTTQSRLQFSQAGASDIRDQSRNWLPGPCYRQQRVSKTSADNNNSEYSWTGATKYHLNGRDSLVNPGPAMASHKDDEEKFFPQSGVLIFGKQGSEKTNVDIEKVMITDESEIAATNPVATEQYGCVATNLQRGYVQAATADVNTQGVLPGMVWQDRDVYLQGPIWAKIPHTDGHFHPSPLMGGFGLKHPPPQILIKNTPVPANPSTTFSAAKFASFITQYSTGQVSVEIEWELQKENSKRWNPEIQYTSNYNKSVNVDFTVDTNGVYSEPRPIGTRYLTRNL

SEQ ID NO: 93 - protein, 533 aa, synthetic construct
  source 1..533: note = Amino acid sequence of VP3 variant
MATGSGAPMADNNEGADGVGNSSGNWHCDSTWMGDRVITTSTRTWALPTYNNHLYKQISSQSGASNDNHYFGYSTPWGYFDFNRFHCHFSPRDWQRLINNNWGFRPKRLNFKLFNIQVKEVTQNDGTTTIANNLTSTVQVFTDSEYQLPYVLGSAHQGCLPPFPADVFMVPQYGYLTLNNGSQAVGRSSFYCLEYFPSQMLRTGNNFTFSYTFEDVPFHSSYAHSQSLDRLMNPLIDQYLYYLSRTNTPSGTTTQSRLQFSQAGASDIRDQSRNWLPGPCYRQQRVSKTSADNNNSEYSWTGATKYHLNGRDSLVNPGPAMASHKDDEEKFFPQSGVLIFGKQGSEKTNVDIEKVMITDEQEVAATNPVATEQWGEVSTNLQRGNEQAATADVNTQGVLPGMVWQDRDVYLQGPIWAKIPHTDGHFHPSPLMGGFGLKHPPPQILIKNTPVPANPSTTFSAAKFASFITQYSTGQVSVEIEWELQKENSKRWNPEIQYTSNYNKSVNVDFTVDTNGVYSEPRPIGTRYLTRNL

SEQ ID NO: 94 - protein, 28 aa, synthetic construct
  source 1..28: note = Wild-type amino acid sequence in a region at positions VP1 561-588
DEEEIRTTNPVATEQYGSVSTNLQRGNR

SEQ ID NO: 95 - protein, 28 aa, synthetic construct
  source 1..28: note = Mutation amino acid sequence in a region at positions VP1 561-588
DEEEIAATNPVATESYGEVATNLQRGNV

SEQ ID NO: 96 - protein, 28 aa, synthetic construct
  source 1..28: note = Mutation amino acid sequence in a region at positions VP1 561-588
DEQEVAATNPVATESWGSVSTNLQRGNT

SEQ ID NO: 97 - protein, 28 aa, synthetic construct
  source 1..28: note = Mutation amino acid sequence in a region at positions VP1 561-588
DESEIRTTNPIATEQWGSVSTNLQNGNR

SEQ ID NO: 98 - protein, 28 aa, synthetic construct
  source 1..28: note = Mutation amino acid sequence in a region at positions VP1 561-588
DEEEIATTNPVATEQWGSVSTNLQRGAT

SEQ ID NO: 99 - protein, 28 aa, synthetic construct
  source 1..28: note = Mutation amino acid sequence in a region at positions VP1 561-588
DESEIATTNPVATESYGEVSTNLQRNPV

SEQ ID NO: 100 - protein, 28 aa, synthetic construct
  source 1..28: note = Mutation amino acid sequence in a region at positions VP1 561-588
DEEEIRTTNPVAYEQYGVVATNLQNSNA

SEQ ID NO: 101 - protein, 28 aa, synthetic construct
  source 1..28: note = Mutation amino acid sequence in a region at positions VP1 561-588
DEAEIATTNPVAAEQYGEVSTNLQNGNR

SEQ ID NO: 102 - protein, 28 aa, synthetic construct
  source 1..28: note = Mutation amino acid sequence in a region at positions VP1 561-588
DEQEVAATNPVATEHYGQVATNLQTGNR

SEQ ID NO: 103 - protein, 28 aa, synthetic construct
  source 1..28: note = Mutation amino acid sequence in a region at positions VP1 561-588
DEEEINTTNPVYTEQYGSVSTNLQRGNI

SEQ ID NO: 104 - protein, 28 aa, synthetic construct
  source 1..28: note = Mutation amino acid sequence in a region at positions VP1 561-588
DEQEVAATNPVADEQYGVVATNLQRGNV

SEQ ID NO: 105 - protein, 28 aa, synthetic construct
  source 1..28: note = Mutation amino acid sequence in a region at positions VP1 561-588
DESEIAATNPVATEQWGSVATNRQRGET

SEQ ID NO: 106 - protein, 28 aa, synthetic construct
  source 1..28: note = Mutation amino acid sequence in a region at positions VP1 561-588
DEQEVAATNPVATEQWGEVSTNLQRSTT

SEQ ID NO: 107 - protein, 28 aa, synthetic construct
  source 1..28: note = Mutation amino acid sequence in a region at positions VP1 561-588
QESEIAATNPVATEQWGVVATNLQNGTR

SEQ ID NO: 108 - protein, 28 aa, synthetic construct
  source 1..28: note = Mutation amino acid sequence in a region at positions VP1 561-588
DESEVAATNPVATEQWGEVSTNNQRGTT

SEQ ID NO: 109 - protein, 28 aa, synthetic construct
  source 1..28: note = Mutation amino acid sequence in a region at positions VP1 561-588
DEEEIRTTNPVATEQYGSVSTNIQHGNR

SEQ ID NO: 110 - protein, 28 aa, synthetic construct
  source 1..28: note = Mutation amino acid sequence in a region at positions VP1 561-588
DEEEIRTTNPVATEQYGSVSTWLQRGNR

SEQ ID NO: 111 - protein, 28 aa, synthetic construct
  source 1..28: note = Mutation amino acid sequence in a region at positions VP1 561-588
DEQEIAATNPVATEQYGEVSTNLQNQNR

SEQ ID NO: 112 - protein, 28 aa, synthetic construct
  source 1..28: note = Mutation amino acid sequence in a region at positions VP1 561-588
QESEIAATNPVATEQWGEVATNLQRGTT

SEQ ID NO: 113 - protein, 28 aa, synthetic construct
  source 1..28: note = Mutation amino acid sequence in a region at positions VP1 561-588
DEWEIRTTNPVATEQYGSVSTNLQRLNR

SEQ ID NO: 114 - protein, 28 aa, synthetic construct
  source 1..28: note = Mutation amino acid sequence in a region at positions VP1 561-588
DEAEIAATNPVATEQWGEVSTNTQNGAR

SEQ ID NO: 115 - protein, 28 aa, synthetic construct
  source 1..28: note = Mutation amino acid sequence in a region at positions VP1 561-588
DEQEVAATNPVATEAYGTVSTNLQRQNT

SEQ ID NO: 116 - protein, 28 aa, synthetic construct
  source 1..28: note = Mutation amino acid sequence in a region at positions VP1 561-588
DEAEIAATNPVATEQYGTVSTNLQTGNQ

SEQ ID NO: 117 - protein, 28 aa, synthetic construct
  source 1..28: note = Mutation amino acid sequence in a region at positions VP1 561-588
DESEIRTTNPVATESYGEVATNLQTGTT

SEQ ID NO: 118 - protein, 28 aa, synthetic construct
  source 1..28: note = Mutation amino acid sequence in a region at positions VP1 561-588
DEAEIATTNPVATEQWGSVSTNLQGGNL

SEQ ID NO: 119 - protein, 28 aa, synthetic construct
  source 1..28: note = Mutation amino acid sequence in a region at positions VP1 561-588
NESEIAATNPVATEQYGVVATNLQNGTV

SEQ ID NO: 120 - protein, 28 aa, synthetic construct
  source 1..28: note = Mutation amino acid sequence in a region at positions VP1 561-588
DESEIRTTNPVATEQWGEVATNLQNGNI

SEQ ID NO: 121 - protein, 28 aa, synthetic construct
  source 1..28: note = Mutation amino acid sequence in a region at positions VP1 561-588
DEAEIAATNPVATEQYGCVASNIQNSNT

SEQ ID NO: 122 - protein, 28 aa, synthetic construct
  source 1..28: note = Mutation amino acid sequence in a region at positions VP1 561-588
DESEIAATNPVAYEQYGSVTTNLQNGNN

SEQ ID NO: 123 - protein, 28 aa, synthetic construct
  source 1..28: note = Mutation amino acid sequence in a region at positions VP1 561-588
DESEIAATNPVATEQYGCVATNLQRGYV

SEQ ID NO: 124 - protein, 28 aa, synthetic construct
  source 1..28: note = Mutation amino acid sequence in a region at positions VP1 561-588
DEQEVAATNPVATEQWGEVSTNLQRGNE

SEQ ID NO: 125 - DNA, 84 bp, synthetic construct
  source 1..84: mol_type = other DNA; note = DNA sequence encoding the mutation amino acid sequence in a region at positions VP1 561-588
gacgaggaggagatcgccgccaccaaccccgtggccaccgagagctacggcgaggtggccaccaacctgcagagaggcaacgtg

SEQ ID NO: 126 - DNA, 84 bp, synthetic construct
  source 1..84: mol_type = other DNA; note = DNA sequence encoding the mutation amino acid sequence in a region at positions VP1 561-588
gacgagcaggaggtggccgccaccaaccccgtggccaccgagagctggggcagcgtgagcaccaacctgcagagaggcaacacc

SEQ ID NO: 127 - DNA, 84 bp, synthetic construct
  source 1..84: mol_type = other DNA; note = DNA sequence encoding the mutation amino acid sequence in a region at positions VP1 561-588
gacgagagcgagatcagaaccaccaaccccatcgccaccgagcagtggggcagcgtgagcaccaacctgcagaacggcaacaga

SEQ ID NO: 128 - DNA, 84 bp, synthetic construct
  source 1..84: mol_type = other DNA; note = DNA sequence encoding the mutation amino acid sequence in a region at positions VP1 561-588
gacgaggaggagatcgccaccaccaaccccgtggccaccgagcagtggggcagcgtgagcaccaacctgcagagaggcgccacc

SEQ ID NO: 129 - DNA, 84 bp, synthetic construct
  source 1..84: mol_type = other DNA; note = DNA sequence encoding the mutation amino acid sequence in a region at positions VP1 561-588
gacgagagcgagatcgccaccaccaaccccgtggccaccgagagctacggcgaggtgagcaccaacctgcagagaaaccccgtg

SEQ ID NO: 130 - DNA, 84 bp, synthetic construct
  source 1..84: mol_type = other DNA; note = DNA sequence encoding the mutation amino acid sequence in a region at positions VP1 561-588
gacgaggaggagatcagaaccaccaaccccgtggcctacgagcagtacggcgtggtggccaccaacctgcagaacagcaacgcc

SEQ ID NO: 131 - DNA, 84 bp, synthetic construct
  source 1..84: mol_type = other DNA; note = DNA sequence encoding the mutation amino acid sequence in a region at positions VP1 561-588
gacgaggccgagatcgccaccaccaaccccgtggccgccgagcagtacggcgaggtgagcaccaacctgcagaacggcaacaga

SEQ ID NO: 132 - DNA, 84 bp, synthetic construct
  source 1..84: mol_type = other DNA; note = DNA sequence encoding the mutation amino acid sequence in a region at positions VP1 561-588
gacgagcaggaggtggccgccaccaaccccgtggccaccgagcactacggccaggtggccaccaacctgcagaccggcaacaga

SEQ ID NO: 133 - DNA, 84 bp, synthetic construct
  source 1..84: mol_type = other DNA; note = DNA sequence encoding the mutation amino acid sequence in a region at positions VP1 561-588
gacgaagaggaaatcaacacaaccaatcccgtgtacacggagcagtatggttctgtatctaccaacctccagagaggcaacatc

SEQ ID NO: 134 - DNA, 84 bp, synthetic construct
  source 1..84: mol_type = other DNA; note = DNA sequence encoding the mutation amino acid sequence in a region at positions VP1 561-588
gacgagcaggaggtggccgccaccaaccccgtggccgacgagcagtacggcgtggtggccaccaacctgcagagaggcaacgtg

SEQ ID NO: 135 - DNA, 84 bp, synthetic construct
  source 1..84: mol_type = other DNA; note = DNA sequence encoding the mutation amino acid sequence in a region at positions VP1 561-588
gacgagagcgagatcgccgccaccaaccccgtggccaccgagcagtggggcagcgtggccaccaacagacagagaggcgagacc

SEQ ID NO: 136 - DNA, 84 bp, synthetic construct
  source 1..84: mol_type = other DNA; note = DNA sequence encoding the mutation amino acid sequence in a region at positions VP1 561-588
gacgagcaggaggtggccgccaccaaccccgtggccaccgagcagtggggcgaggtgagcaccaacctgcagagaagcaccacc

SEQ ID NO: 137 - DNA, 84 bp, synthetic construct
  source 1..84: mol_type = other DNA; note = DNA sequence encoding the mutation amino acid sequence in a region at positions VP1 561-588
caggagagcgagatcgccgccaccaaccccgtggccaccgagcagtggggcgtggtggccaccaacctgcagaacggcaccaga

SEQ ID NO: 138 - DNA, 84 bp, synthetic construct
  source 1..84: mol_type = other DNA; note = DNA sequence encoding the mutation amino acid sequence in a region at positions VP1 561-588
gacgagagcgaggtggccgccaccaaccccgtggccaccgagcagtggggcgaggtgagcaccaacaaccagagaggcaccacc

SEQ ID NO: 139 - DNA, 84 bp, synthetic construct
  source 1..84: mol_type = other DNA; note = DNA sequence encoding the mutation amino acid sequence in a region at positions VP1 561-588
gacgaagaggaaatcaggacaaccaatcccgtggctacggagcagtatggttctgtatctaccaacatccagcacggcaacaga

SEQ ID NO: 140 - DNA, 84 bp, synthetic construct
  source 1..84: mol_type = other DNA; note = DNA sequence encoding the mutation amino acid sequence in a region at positions VP1 561-588
gacgaagaggaaatcaggacaaccaatcccgtggctacggagcagtatggttctgtatctacctggctccagagaggcaacaga

SEQ ID NO: 141 - DNA, 84 bp, synthetic construct
  source 1..84: mol_type = other DNA; note = DNA sequence encoding the mutation amino acid sequence in a region at positions VP1 561-588
gacgagcaggagatcgccgccaccaaccccgtggccaccgagcagtacggcgaggtgagcaccaacctgcagaaccagaacaga

SEQ ID NO: 142 - DNA, 84 bp, synthetic construct
  source 1..84: mol_type = other DNA; note = DNA sequence encoding the mutation amino acid sequence in a region at positions VP1 561-588
caggagagcgagatcgccgccaccaaccccgtggccaccgagcagtggggcgaggtggccaccaacctgcagagaggcaccacc

SEQ ID NO: 143 - DNA, 84 bp, synthetic construct
  source 1..84: mol_type = other DNA; note = DNA sequence encoding the mutation amino acid sequence in a region at positions VP1 561-588
gacgaatgggaaatcaggacaaccaatcccgtggctacggagcagtatggttctgtatctaccaacctccagagactgaacaga

SEQ ID NO: 144 - DNA, 84 bp, synthetic construct
  source 1..84: mol_type = other DNA; note = DNA sequence encoding the mutation amino acid sequence in a region at positions VP1 561-588
gacgaggccgagatcgccgccaccaaccccgtggccaccgagcagtggggcgaggtgagcaccaacacccagaacggcgccaga

SEQ ID NO: 145 - DNA, 84 bp, synthetic construct
  source 1..84: mol_type = other DNA; note = DNA sequence encoding the mutation amino acid sequence in a region at positions VP1 561-588
gacgagcaggaggtggccgccaccaaccccgtggccaccgaggcctacggcaccgtgagcaccaacctgcagagacagaacacc

SEQ ID NO: 146 - DNA, 84 bp, synthetic construct
  source 1..84: mol_type = other DNA; note = DNA sequence encoding the mutation amino acid sequence in a region at positions VP1 561-588
gacgaggccgagatcgccgccaccaaccccgtggccaccgagcagtacggcaccgtgagcaccaacctgcagaccggcaaccag

SEQ ID NO: 147 - DNA, 84 bp, synthetic construct
  source 1..84: mol_type = other DNA; note = DNA sequence encoding the mutation amino acid sequence in a region at positions VP1 561-588
gacgagagcgagatcagaaccaccaaccccgtggccaccgagagctacggcgaggtggccaccaacctgcagaccggcaccacc

SEQ ID NO: 148 - DNA, 84 bp, synthetic construct
  source 1..84: mol_type = other DNA; note = DNA sequence encoding the mutation amino acid sequence in a region at positions VP1 561-588
gacgaggccgagatcgccaccaccaaccccgtggccaccgagcagtggggcagcgtgagcaccaacctgcagggcggcaacctg

SEQ ID NO: 149 - DNA, 84 bp, synthetic construct
  source 1..84: mol_type = other DNA; note = DNA sequence encoding the mutation amino acid sequence in a region at positions VP1 561-588
aacgagagcgagatcgccgccaccaaccccgtggccaccgagcagtacggcgtggtggccaccaacctgcagaacggcaccgtg

SEQ ID NO: 150 - DNA, 84 bp, synthetic construct
  source 1..84: mol_type = other DNA; note = DNA sequence encoding the mutation amino acid sequence in a region at positions VP1 561-588
gacgagagcgagatcagaaccaccaaccccgtggccaccgagcagtggggcgaggtggccaccaacctgcagaacggcaacatc

SEQ ID NO: 151 - DNA, 84 bp, synthetic construct
  source 1..84: mol_type = other DNA; note = DNA sequence encoding the mutation amino acid sequence in a region at positions VP1 561-588
gacgaggccgagatcgccgccaccaaccccgtggccaccgagcagtacggctgcgtggccagcaacatccagaacagcaacacc

SEQ ID NO: 152 - DNA, 84 bp, synthetic construct
  source 1..84: mol_type = other DNA; note = DNA sequence encoding the mutation amino acid sequence in a region at positions VP1 561-588
gacgagagcgagatcgccgccaccaaccccgtggcctacgagcagtacggcagcgtgaccaccaacctgcagaacggcaacaac

SEQ ID NO: 153 - DNA, 84 bp, synthetic construct
  source 1..84: mol_type = other DNA; note = DNA sequence encoding the mutation amino acid sequence in a region at positions VP1 561-588
gacgagagcgagatcgccgccaccaaccccgtggccaccgagcagtacggctgcgtggccaccaacctgcagagaggctacgtg

SEQ ID NO: 154 - DNA, 84 bp, synthetic construct
  source 1..84: mol_type = other DNA; note = DNA sequence encoding the mutation amino acid sequence in a region at positions VP1 561-588
gacgagcaggaggtggccgccaccaaccccgtggccaccgagcagtggggcgaggtgagcaccaacctgcagagaggcaacgag

SEQ ID NO: 155 - DNA, 21 bp, synthetic construct
  source 1..21: mol_type = other DNA; note = DNA sequence of forward primer
gagcggggttctcatctttgg

SEQ ID NO: 156 - DNA, 20 bp, synthetic construct
  source 1..20: mol_type = other DNA; note = DNA sequence of reverse primer
tgcctggaagaacgccttgt